European Patent Application EP 4 793 347 A1, published August 19, 2026. Title: Variants of metazoan fatty acid synthase for the production of fatty acids, aldehydes and alcohols. Applicant: Johann Wolfgang Goethe-Universitaet Frankfurt am Main. The sequence listing filed with the application follows.

SEQUENCE LISTING (35 sequences)

SEQ ID NO: 1 - protein, 406 aa, Mus musculus
MEEVVIAGMSGKLPESENLQEFWANLIGGVDMVTDDDRRWKAGLYGLPKRSGKLKDLSKFDASFFGVHPKQAHTMDPQLRLLLEVSYEAIVDGGINPASLRGTNTGVWVGVSGSEASEALSRDPETLLGYSMVGCQRAMMANRLSFFFDFKGPSIALDTACSSSLLALQNAYQAIRSGECPAALVGGINLLLKPNTSVQFMKLGMLSPDGTCRSFDDSGSGYCRSEAVVAVLLTKKSLARRVYATILNAGTNTDGSKEQGVTFPSGEVQEQLICSLYQPAGLAPESLEYIEAHGTGTKVGDPQELNGITRSLCAFRQAPLLIGSTKSNMGHPEPASGLAALTKVLLSLEHGVWAPNLHFHNPNPEIPALLDGRLQVVDRPLPVRGGNVGINSFGFGGSNVHVILQP

SEQ ID NO: 2 - protein, 182 aa, Escherichia coli
ADTLLILGDSLSAGYRMSASAAWPALLNDKWQSKTSVVNASISGDTSQQGLARLPALLKQHQPRWVLVELGGNDGLRGFQPQQTEQTLRQILQDVKAANAEPLLMQIRLPANYGRRYNEAFSAIYPKLAKEFDVPLLPFFMEEVYLKPQWMQDDGIHPNRDAQPFIADWMAKQLQPLVNHDS

SEQ ID NO: 3 - protein, 450 aa, Mycobacterium phlei
TARRPGDGRPTFAGVHGDDAAEVHARDLTLDRFLDDATLAAATALPGPAPEIRTVLLTGATGFLGRYLALEWLERMAMVGGTLICLVRGRDDAAARARLDQIFDSGDPELLRHYRELADRHLEVIAGDKSDAVLGLDRRTWQRLADTVDLIVDPAALVNHVLPYRELFGPNVVGTAELIRLALTGRLKPYLYTSTIAVGAGIAPGQFTEDADIRQISATRTLDDSYANGYATSKWAGEVLLREAHDLCGLPVAVFRCDMILADTSYAGQLNVPDMFTRLILSLVATGIAPLSFYELDAAGHRQRAHYDGLPVEFVAEAVSALGLDVAEDGGFATYHVMNPYDDGIGLDEFVDWLTGAGYPIERVNDYGTWFQRFETAIRGLPERQRQASLLPLLHNYQRPQPPIRGSAAPTDRFRSAVQDAKIGPDKDIPHITPEVIVKYVTDLRLLGLL

SEQ ID NO: 4 - protein, 442 aa, Mycobacterium smegmatis
AQRTAGDRRPSFTTVHGADATEIRASELTLDKFIDAETLRAAPGLPKVTTEPRTVLLSGANGWLGRFLTLQWLERLAPVGGTLITIVRGRDDAAARARLTQAYDTDPELSRRFAELADRHLRVVAGDIGDPNLGLTPEIWHRLAAEVDLVVHPAALVNHVLPYRQLFGPNVVGTAEVIKLALTERIKPVTYLSTVSVAMGIPDFEEDGDIRTVSPVRPLDGGYANGYGNSKWAGEVLLREAHDLCGLPVATFRSDMILAHPRYRGQVNVPDMFTRLLLSLLITGVAPRSFYIGDGERPRAHYPGLTVDFVAEAVTTLGAQQREGYVSYDVMNPHDDGISLDVFVDWLIRAGHPIDRVDDYDDWVRRFETALTALPEKRRAQTVLPLLHAFRAPQAPLRGAPEPTEVFHAAVRTAKVGPGDIPHLDEALIDKYIRDLREFGLI

SEQ ID NO: 5 - protein, 445 aa, Nocardia otitidiscaviarum
SERDSGSRPTAATVHGDDGLLRADDLALEAFLDPATLDAAAHLPSALEPPRTVLLTGANGYLGRFLALEWLQRLDVSGGTLICLIRGSDADSARRRLDAVFATGDPELEAHYRELAERRLRVLPGDIGEPNLGLREQDWRDLAETVDLIVHPAALVNHVLPYAQLFGPNVVGTAEVIRLALTSRLKPVTYLSTVAVSAGIDPETFTEDGDIREISPVRRLDDGYANGYGNSKWAGEVLLRNAHDRFGLPVAVFRSDMILAHSRYAGQLNVPDMFTRLLLSVLATGLAPGSFHDAHGERHRAHYDGLPADFTAAAVTTLGSRVTSGYETYDVLNPHDDGISLDTFVDWLIEAGHPIDRIDDYAEWFARFDTALRALPEHQRQHSLLPLLHAYRRPTPPLHGVALPAKHFRAAVQQAKLGPDGDIPHVTRELIEKYASDLRLLGLIQ

SEQ ID NO: 6 - protein, 2394 aa, synthetic construct
MEEVVIAGMSGKLPESENLQEFWANLIGGVDMVTDDDRRWKAGLYGLPKRSGKLKDLSKFDASFFGVHPKQAHTMDPQLRLLLEVSYEAIVDGGINPASLRGTNTGVWVGVSGSEASEALSRDPETLLGYSMVGCQRAMMANRLSFFFDFKGPSIALDTACSSSLLALQNAYQAIRSGECPAALVGGINLLLKPNTSVQFMKLGMLSPDGTCRSFDDSGSGYCRSEAVVAVLLTKKSLARRVYATILNAGTNTDGSKEQGVTFPSGEVQEQLICSLYQPAGLAPESLEYIEAHGTGTKVGDPQELNGITRSLCAFRQAPLLIGSTKSNMGHPEPASGLAALTKVLLSLEHGVWAPNLHFHNPNPEIPALLDGRLQVVDRPLPVRGGNVGINSFGFGGSNVHVILQPNTRQAPAPTAHAALPHLLHASGRTLEAVQDLLEQGRQHSQDLAFVSMLNDIAATPTAAMPFRGYTVLGVEGRVQEVQQVSTNKRPLWFICSGMGTQWRGMGLSLMRLDSFRESILRSDEAVKPLGVKVSDLLLSTDERTFDDIVHAFVSLTAIQIALIDLLTSVGLKPDGIIGHSLGEVACGYADGCLSQREAVLAAYWRGQCIKDAHLPPGSMAAVGLSWEECKQRCPAGVVPACHNSEDTVTISGPQAAVNEFVEQLKQEGVFAKEVRTGGLAFHSYFMEGIAPTLLQALKKVIREPRPRSARWLSTSIPEAQWQSSLARTSSAEYNVNNLVSPVLFQEALWHIPEHAVVLEIAPHALLQAVLKRGVKSSCTIIPLMKRDHKDNLEFFLTNLGKVHLTGINVNPNALFPPVEFPAPRGTPLISPHIKWDHSQTWDVPVAEDFPNGSSSSSATVYSIDASPESPDHYLVDHCIDGRVIFPGTGYLCLVWKTLARSLGLSLEETPVVFENVSFHQATILPKTGTVALEVRLLEASHAFEVSDTGNLIVSGKVYLWEDPNSKLFDHPEVPTPPESASVSRLTQGEVYKELRLRGYDYGPQFQGICEATLEGEQGKLLWKDNWVTFMDTMLQVSILGSSQQSLQLPTRVTAIYIDPATHRQKVYRLKEDTQVADVTTSRCLGITVSGGIHISRLQTTATSRRQQEQLVPTLEKFVFTPHMEAECLSESTALQKELQLCKGLARALQTKATQQGLKAAMLGQEDPPQHGLPRLLAAACQLQLNGNLQLELGEALAQERLLLPEDPLISGLLNSQALKACVDTALENLSTLKMKVAEVLAGEGHLYSRIPALLNTQPMLQLEYTATDRHPQALKDVQTKLQQHDVAQGQWNPSDPAPSSLGALDLLVCNCALATLGDPALALDNMVAALKEGGFLLVHTVLKGHALGETLACLPSEVQPAPSLLSQEEWESLFSRKALHLVGLKRSFYGTALFLCRRAIPQEKPIFLSVEDTSFQWVDSLKSTLATSSSQPVWLTAMDCPTSGVVGLVNCLRKEPGGHRIRCILLSNLSNTSHAPKLDPGSPELQQVLKHDLVMNVYRDGAWGAFRHFQLEQDKPKEQTAHAFVNVLTRGDLASIRWVSSPLKHTQPSSSGAQLCTVYYASLNFRDIMLATGKLSPDAIPGKWASRDCMLGMEFSGRDRCGRRVMGLVPAEGLATSVLLSSDFLWDVPSSWTLEEAASVPVVYTTAYYSLVVRGRIQRGETVLIHSGSGGVGQAAISIALSLGCRVFTTVGSAEKRAYLQARFPQLDDTSFANSRDTSFEQHVLLHTGGKGVDLVLNSLAEEKLQASVRCLAQHGRFLEIGKFDLSNNHPLGMAIFLKNVTFHGILLDALFEEANDSWREVAALLKAGIRDGVVKPLKCTVFPKAQVEDAFRYMAQGKHIGKVLVQVREEEPEAVLPGAQPTLISAISKTFCPAHKSYIITGGLGGFGLELARWLVLRGAQRLVLTSRSGIRTGYQAKHIREWRRQGIQVLVSTSNVSSLEGARALIAEATKLGPVGGVFNLAMVLRDAMLENQTPELFQDVNKPKYNGTLNLDRATREACPELDYFVAFSSVSCGRGNAGQTNYGFANSTMERICEQRRHDGLPGLAVQWGAIGDVGIVLEAMGTNDTVIGGTLPQRISSCMEVLDLFLNQPHAVLSSFVLAEKKAVAHGDGDTQRDLVKAVAHILGIRDLAGINLDSTLADLGLDSLMGVEVRQILEREHDLVLPMREVRQLTLRKLQEMSSKTDSATDTTAPKSRSDTSLKQNQAAAADTLLILGDSLSAGYRMSASAAWPALLNDKWQSKTSVVNASISGDTSQQGLARLPALLKQHQPRWVLVELGGNDGLRGFQPQQTEQTLRQILQDVKAANAEPLLMQIRLPANYGRRYNEAFSAIYPKLAKEFDVPLLPFFMEEVYLKPQWMQDDGIHPNRDAQPFIADWMAKQLQPLVNHDS

SEQ ID NO: 7 - protein, 2394 aa, synthetic construct
MEEVVIAGMSGKLPESENLQEFWANLIGGVDMVTDDDRRWKAGLYGLPKRSGKLKDLSKFDASFFGVHPKQAHTMDPQLRLLLEVSYEAIVDGGINPASLRGTNTGVWVGVSGSEASEALSRDPETLLGYSMVGCQRAMMANRLSFFFDFKGPSIALDTACSSSLLALQNAYQAIRSGECPAALVGGINLLLKPNTSVQFMKLGMLSPDGTCRSFDDSGSGYCRSEAVVAVLLTKKSLARRVYATILNAGTNTDGSKEQGVTFPSGEVQEQLICSLYQPAGLAPESLEYIEAHGTGTKVGDPQELNGITRSLCAFRQAPLLIGSTKSNMGHPEPASGLAALTKVLLSLEHGVWAPNLHFHNPNPEIPALLDGRLQVVDRPLPVRGGNVGINSFGFGGSNVHVILQPNTRQAPAPTAHAALPHLLHASGRTLEAVQDLLEQGRQHSQDLAFVSMLNDIAATPTAAMPFRGYTVLGVEGRVQEVQQVSTNKRPLWFICSGMGTQWRGMGLSLMRLDSFRESILRSDEAVKPLGVKVSDLLLSTDERTFDDIVHAFVSLTAIQIALIDLLTSVGLKPDGIIGHSLGEVACGYADGCLSQREAVLAAYWRGQCIKDAHLPPGSMAAVGLSWEECKQRCPAGVVPACHNSEDTVTISGPQAAVNEFVEQLKQEGVFAKEVRTGGLAFHSYFMEGIAPTLLQALKKVIREPRPRSARWLSTSIPEAQWQSSLARTSSAEYNVNNLVSPVLFQEALWHIPEHAVVLEIAPHALLQAVLKRGVKSSCTIIPLMKRDHKDNLEFFLTNLGKVHLTGINVNPNALFPPVEFPAPRGTPLISPHIKWDHSQTWDVPVAEDFPNGSSSSSATVYSIDASPESPDHYLVDHCIDGRVIFPGTGYLCLVWKTLARSLGLSLEETPVVFENVSFHQATILPKTGTVALEVRLLEASHAFEVSDTGNLIVSGKVYLWEDPNSKLFDHPEVPTPPESASVSRLTQGEVYKELRLRGYDYGPQFQGICEATLEGEQGKLLWKDNWVTFMDTMLQVSILGSSQQSLQLPTRVTAIYIDPATHRQKVYRLKEDTQVADVTTSRCLGITVSGGIHISRLQTTATSRRQQEQLVPTLEKFVFTPHMEAECLSESTALQKELQLCKGLARALQTKATQQGLKAAMLGQEDPPQHGLPRLLAAACQLQLNGNLQLELGEALAQERLLLPEDPLISGLLNSQALKACVDTALENLSTLKMKVAEVLAGEGHLYSRIPALLNTQPMLQLEYTATDRHPQALKDVQTKLQQHDVAQGQWNPSDPAPSSLGALDLLVCNCALATLGDPALALDNMVAALKEGGFLLVHTVLKGHALGETLACLPSEVQPAPSLLSQEEWESLFSRKALHLVGLKRSFYGTALFLCRRAIPQEKPIFLSVEDTSFQWVDSLKSTLATSSSQPVWLTAMDCPTSGVVGLVNCLRKEPGGHRIRCILLSNLSNTSHAPKLDPGSPELQQVLKHDLVMNVYRDGAWGAFRHFQLEQDKPKEQTAHAFVNVLTRGDLASIRWVSSPLKHTQPSSSGAQLCTVYYASLNFRDIMLATGKLSPDAIPGKWASRDCMLGMEFSGRDRCGRRVMGLVPAEGLATSVLLSSDFLWDVPSSWTLEEAASVPVVYTTAYYSLVVRGRIQRGETVLIHSGSGGVGQAAISIALSLGCRVFTTVGSAEKRAYLQARFPQLDDTSFANSRDTSFEQHVLLHTGGKGVDLVLNSLAEEKLQASVRCLAQHGRFLEIGKFDLSNNHPLGMAIFLKNVTFHGILLDALFEEANDSWREVAALLKAGIRDGVVKPLKCTVFPKAQVEDAFRYMAQGKHIGKVLVQVREEEPEAVLPGAQPTLISAISKTFCPAHKSYIITGGLGGFGLELARWLVLRGAQRLVLTSRSGIRTGYQAKHIREWRRQGIQVLVSTSNVSSLEGARALIAEATKLGPVGGVFNLAMVLRDAMLENQTPELFQDVNKPKYNGTLNLDRATREACPELDYFVAFSSVSCGRGNAGQTNYGFANSTMERICEQRRHDGLPGLAVQWGAIGDVGIVLEAMGTNDTVIGGTLPQRISSCMEVLDLFLNQPHAVLSSFVLAEKKAVAHGDGDTQRDLVKAVAHILGIRDLAGINLDSTLADLGLDSLMGVEVRQILEREHDLVLPMREVRQLTLRKLQEMSSKTDSATDTTAPKSRSDTSLKQNQAAAADTLLILGDSLSAGYRMSASAAWPALLNDKWQSKTSVVNASISGDTSQQGLARLPALLKQHQPRWVLVELGGNDGLRGFQPQQTEQTLRQILQDVKAANAEPLLMQIRPPANYGRRYNEAFSAIYPKLAKEFDVPLLPFFMEEVYLKPQWMQDDGIHPNRDAQPFIADWMAKQLQPLVNHDS

SEQ ID NO: 8 - protein, 2394 aa, synthetic construct
MEEVVIAGMSGKLPESENLQEFWANLIGGVDMVTDDDRRWKAGLYGLPKRSGKLKDLSKFDASFFGVHPKQAHTMDPQLRLLLEVSYEAIVDGGINPASLRGTNTGVWVGVSGSEASEALSRDPETLLGYSMVGCQRAMMANRLSFFFDFKGPSIALDTACSSSLLALQNAYQAIRSGECPAALVGGINLLLKPNTSVQFMKLGMLSPDGTCRSFDDSGSGYCRSEAVVAVLLTKKSLARRVYATILNAGTNTDGSKEQGVTFPSGEVQEQLICSLYQPAGLAPESLEYIEAHGTGTKVGDPQELNGITRSLCAFRQAPLLIGSTKSNMGHPEPASGLAALTKVLLSLEHGVWAPNLHFHNPNPEIPALLDGRLQVVDRPLPVRGGNVGINSFGFGGSNVHVILQPNTRQAPAPTAHAALPHLLHASGRTLEAVQDLLEQGRQHSQDLAFVSMLNDIAATPTAAMPFRGYTVLGVEGRVQEVQQVSTNKRPLWFICSGMGTQWRGMGLSLMRLDSFRESILRSDEAVKPLGVKVSDLLLSTDERTFDDIVHAFVSLTAIQIALIDLLTSVGLKPDGIIGHSLGEVACGYADGCLSQREAVLAAYWRGQCIKDAHLPPGSMAAVGLSWEECKQRCPAGVVPACHNSEDTVTISGPQAAVNEFVEQLKQEGVFAKEVRTGGLAFHSYFMEGIAPTLLQALKKVIREPRPRSARWLSTSIPEAQWQSSLARTSSAEYNVNNLVSPVLFQEALWHIPEHAVVLEIAPHALLQAVLKRGVKSSCTIIPLMKRDHKDNLEFFLTNLGKVHLTGINVNPNALFPPVEFPAPRGTPLISPHIKWDHSQTWDVPVAEDFPNGSSSSSATVYSIDASPESPDHYLVDHCIDGRVIFPGTGYLCLVWKTLARSLGLSLEETPVVFENVSFHQATILPKTGTVALEVRLLEASHAFEVSDTGNLIVSGKVYLWEDPNSKLFDHPEVPTPPESASVSRLTQGEVYKELRLRGYDYGPQFQGICEATLEGEQGKLLWKDNWVTFMDTMLQVSILGSSQQSLQLPTRVTAIYIDPATHRQKVYRLKEDTQVADVTTSRCLGITVSGGIHISRLQTTATSRRQQEQLVPTLEKFVFTPHMEAECLSESTALQKELQLCKGLARALQTKATQQGLKAAMLGQEDPPQHGLPRLLAAACQLQLNGNLQLELGEALAQERLLLPEDPLISGLLNSQALKACVDTALENLSTLKMKVAEVLAGEGHLYSRIPALLNTQPMLQLEYTATDRHPQALKDVQTKLQQHDVAQGQWNPSDPAPSSLGALDLLVCNCALATLGDPALALDNMVAALKEGGFLLVHTVLKGHALGETLACLPSEVQPAPSLLSQEEWESLFSRKALHLVGLKRSFYGTALFLCRRAIPQEKPIFLSVEDTSFQWVDSLKSTLATSSSQPVWLTAMDCPTSGVVGLVNCLRKEPGGHRIRCILLSNLSNTSHAPKLDPGSPELQQVLKHDLVMNVYRDGAWGAFRHFQLEQDKPKEQTAHAFVNVLTRGDLASIRWVSSPLKHTQPSSSGAQLCTVYYASLNFRDIMLATGKLSPDAIPGKWASRDCMLGMEFSGRDRCGRRVMGLVPAEGLATSVLLSSDFLWDVPSSWTLEEAASVPVVYTTAYYSLVVRGRIQRGETVLIHSGSGGVGQAAISIALSLGCRVFTTVGSAEKRAYLQARFPQLDDTSFANSRDTSFEQHVLLHTGGKGVDLVLNSLAEEKLQASVRCLAQHGRFLEIGKFDLSNNHPLGMAIFLKNVTFHGILLDALFEEANDSWREVAALLKAGIRDGVVKPLKCTVFPKAQVEDAFRYMAQGKHIGKVLVQVREEEPEAVLPGAQPTLISAISKTFCPAHKSYIITGGLGGFGLELARWLVLRGAQRLVLTSRSGIRTGYQAKHIREWRRQGIQVLVSTSNVSSLEGARALIAEATKLGPVGGVFNLAMVLRDAMLENQTPELFQDVNKPKYNGTLNLDRATREACPELDYFVAFSSVSCGRGNAGQTNYGFANSTMERICEQRRHDGLPGLAVQWGAIGDVGIVLEAMGTNDTVIGGTLPQRISSCMEVLDLFLNQPHAVLSSFVLAEKKAVAHGDGDTQRDLVKAVAHILGIRDLAGINLDSTLADLGLDSLMGVEVRQILEREHDLVLPMREVRQLTLRKLQEMSSKTDSATDTTAPKSRSDTSLKQNQAAAADTLLILGDSLSAGYRMSASAAWPALLNDKWQSKTSVVNASISGDTSQQGLARLPALLKQHQPRWVLVELGGNDGLRGFQPQQTEQTLRQILQDVKAANAEPLLMQIRLPANYGRRYNEAFSAIYPKLAKEFDVPLLPFFLDEVGKKPQWMQDDGIHPNRDAQPFIADWMAKQLQPLVNHDS

SEQ ID NO: 9 - protein, 2504 aa, synthetic construct
MEEVVIAGMSGKLPESENLQEFWANLIGGVDMVTDDDRRWKAGLYGLPKRSGKLKDLSKFDASFFGVHPKQAHTMDPQLRLLLEVSYEAIVDGGINPASLRGTNTGVWVGVSSSEASEALSRDPETLLGYSMVGCQRAMMANRLSFFFDFKGPSIALDTACSSSLLALQNAYQAIRSGECPAALVGGINLLLKPNTSVQFMKLGMLSPDGTCRSFDDSGSGYCRSEAVVAVLLTKKSLARRVYATILNAGTNTDGSKEQGVTFPSGEVQEQLICSLYQPAGLAPESLEYIEAHGTGTKVGDPQELNGITRSLCAFRQAPLLIGSTKSNMGHPEPASGLAALTKVLLSLEHGVWAPNLHFHNPNPEIPALLDGRLQVVDRPLPVRGGNVGINSFGFGGSNVHVILQPNTRQAPAPTAHAALPHLLHASGRTLEAVQDLLEQGRQHSQDLAFVSMLNDIAATPTAAMPFRGYTVLGVEGRVQEVQQVSTNKRPLWFICSGMGTQWRGMGLSLMRLDSFRESILRSDEAVKPLGVKVSDLLLSTDERTFDDIVHAFVSLTAIQIALIDLLTSVGLKPDGIIGHSLGEVACGYADGCLSQREAVLAAYWRGQCIKDAHLPPGSMAAVGLSWEECKQRCPAGVVPACHNSEDTVTISGPQAAVNEFVEQLKQEGVFAKEVRTGGLAFHSYFMEGIAPTLLQALKKVIREPRPRSARWLSTSIPEAQWQSSLARTSSAEYNVNNLVSPVLFQEALWHIPEHAVVLEIAPHALLQAVLKRGVKSSCTIIPLMKRDHKDNLEFFLTNLGKVHLTGINVNPNALFPPVEFPAPRGTPLISPHIKWDHSQTWDVPVAEDFPNGSSSSSATVYSIDASPESPDHYLVDHCIDGRVIFPGTGYLCLVWKTLARSLGLSLEETPVVFENVSFHQATILPKTGTVALEVRLLEASHAFEVSDTGNLIVSGKVYLWEDPNSKLFDHPEVPTPPESASVSRLTQGEVYKELRLRGYDYGPQFQGICEATLEGEQGKLLWKDNWVTFMDTMLQVSILGSSQQSLQLPTRVTAIYIDPATHRQKVYRLKEDTQVADVTTSRCLGITVSGGIHISRLQTTATSRRQQEQLVPTLEKFVFTPHMEAECLSESTALQKELQLCKGLARALQTKATQQGLKAAMLGQEDPPQHGLPRLLAAACQLQLNGNLQLELGEALAQERLLLPEDPLISGLLNSQALKACVDTALENLSTLKMKVAEVLAGEGHLYSRIPALLNTQPMLQLEYTATDRHPQALKDVQTKLQQHDVAQGQWNPSDPAPSSLGALDLLVCNCALATLGDPALALDNMVAALKEGGFLLVHTVLKGHALGETLACLPSEVQPAPSLLSQEEWESLFSRKALHLVGLKRSFYGTALFLCRRAIPQEKPIFLSVEDTSFQWVDSLKSTLATSSSQPVWLTAMDCPTSGVVGLVNCLRKEPGGHRIRCILLSNLSNTSHAPKLDPGSPELQQVLKHDLVMNVYRDGAWGAFRHFQLEQDKPKEQTAHAFVNVLTRGDLASIRWVSSPLKHTQPSSSGAQLCTVYYASLNFRDIMLATGKLSPDAIPGKWASRDCMLGMEFSGRDRCGRRVMGLVPAEGLATSVLLSSDFLWDVPSSWTLEEAASVPVVYTTAYYSLVVRGRIQRGETVLIHSGSGGVGQAAISIALSLGCRVFTTVGSAEKRAYLQARFPQLDDTSFANSRDTSFEQHVLLHTGGKGVDLVLNSLAEEKLQASVRCLAQHGRFLEIGKFDLSNNHPLGMAIFLKNVTFHGILLDALFEEANDSWREVAALLKAGIRDGVVKPLKCTVFPKAQVEDAFRYMAQGKHIGKVLVQVREEEPEAVLPGAQPTLISAISKTFCPAHKSYIITGGLGGFGLELARWLVLRGAQRLVLTSRSGIRTGYQAKHIREWRRQGIQVLVSTSNVSSLEGARALIAEATKLGPVGGVFNLAMVLRDAMLENQTPELFQDVNKPKYNGTLNLDRATREACPELDYFVAFSSVSCGRGNAGQTNYGFANSTMERICEQRRHDGLPGLAVQWGAIGDVGIVLEAMGTNDTVIGGTLPQRISSCMEVLDLFLNQPHAVLSSFVLAEKKAVAHGDGDTQRDLVKAVAHILGIRDLAGINLDSTLADLGLDSLMGVEVRQILEREHDLVLPMREVRQLTLRKLQEMSSKTDSATDTTAPKSRSDTSLKQNQLNLSTLLVNPEGPTLTQLNSVQSSERPLFLVHPIEGSTTVFHSLAAKLSVPTYGLQCTQAAPLDSIPNLAAYYIDCIKQVQPEGPYRIAGYSFGACVAFEMCSQLQAQQGPAPTHNNLFLFDGSHTYVLAYTQSYRAKMTPGCEAEAEAEALCFFIKQFLDVEHSKVLEALLPLKSLEDRVAASVDLITKSHHSLDRRELSFAAVSFYHKLRAADQYKPKAKYHGNVTLLRAKTGGTYGEDLGADYNLSQVCDGKVSVHIIEGDHRTLLEGSGLESIINIIHSSLAEPRVSVREG

SEQ ID NO: 10 - protein, 2394 aa, synthetic construct
MEEVVIAGMSGKLPESENLQEFWANLIGGVDMVTDDDRRWKAGLYGLPKRSGKLKDLSKFDASFFGVHPKQAHTMDPQLRLLLEVSYEAIVDGGINPASLRGTNTGVWVGVSSSEASEALSRDPETLLGYSMVGCQRAMMANRLSFFFDFKGPSIALDTACSSSLLALQNAYQAIRSGECPAALVGGINLLLKPNTSVQFMKLGMLSPDGTCRSFDDSGSGYCRSEAVVAVLLTKKSLARRVYATILNAGTNTDGSKEQGVTFPSGEVQEQLICSLYQPAGLAPESLEYIEAHGTGTKVGDPQELNGITRSLCAFRQAPLLIGSTKSNMGHPEPASGLAALTKVLLSLEHGVWAPNLHFHNPNPEIPALLDGRLQVVDRPLPVRGGNVGINSFGFGGSNVHVILQPNTRQAPAPTAHAALPHLLHASGRTLEAVQDLLEQGRQHSQDLAFVSMLNDIAATPTAAMPFRGYTVLGVEGRVQEVQQVSTNKRPLWFICSGMGTQWRGMGLSLMRLDSFRESILRSDEAVKPLGVKVSDLLLSTDERTFDDIVHAFVSLTAIQIALIDLLTSVGLKPDGIIGHSLGEVACGYADGCLSQREAVLAAYWRGQCIKDAHLPPGSMAAVGLSWEECKQRCPAGVVPACHNSEDTVTISGPQAAVNEFVEQLKQEGVFAKEVRTGGLAFHSYFMEGIAPTLLQALKKVIREPRPRSARWLSTSIPEAQWQSSLARTSSAEYNVNNLVSPVLFQEALWHIPEHAVVLEIAPHALLQAVLKRGVKSSCTIIPLMKRDHKDNLEFFLTNLGKVHLTGINVNPNALFPPVEFPAPRGTPLISPHIKWDHSQTWDVPVAEDFPNGSSSSSATVYSIDASPESPDHYLVDHCIDGRVIFPGTGYLCLVWKTLARSLGLSLEETPVVFENVSFHQATILPKTGTVALEVRLLEASHAFEVSDTGNLIVSGKVYLWEDPNSKLFDHPEVPTPPESASVSRLTQGEVYKELRLRGYDYGPQFQGICEATLEGEQGKLLWKDNWVTFMDTMLQVSILGSSQQSLQLPTRVTAIYIDPATHRQKVYRLKEDTQVADVTTSRCLGITVSGGIHISRLQTTATSRRQQEQLVPTLEKFVFTPHMEAECLSESTALQKELQLCKGLARALQTKATQQGLKAAMLGQEDPPQHGLPRLLAAACQLQLNGNLQLELGEALAQERLLLPEDPLISGLLNSQALKACVDTALENLSTLKMKVAEVLAGEGHLYSRIPALLNTQPMLQLEYTATDRHPQALKDVQTKLQQHDVAQGQWNPSDPAPSSLGALDLLVCNCALATLGDPALALDNMVAALKEGGFLLVHTVLKGHALGETLACLPSEVQPAPSLLSQEEWESLFSRKALHLVGLKRSFYGTALFLCRRAIPQEKPIFLSVEDTSFQWVDSLKSTLATSSSQPVWLTAMDCPTSGVVGLVNCLRKEPGGHRIRCILLSNLSNTSHAPKLDPGSPELQQVLKHDLVMNVYRDGAWGAFRHFQLEQDKPKEQTAHAFVNVLTRGDLASIRWVSSPLKHTQPSSSGAQLCTVYYASLNFRDIMLATGKLSPDAIPGKWASRDCMLGMEFSGRDRCGRRVMGLVPAEGLATSVLLSSDFLWDVPSSWTLEEAASVPVVYTTAYYSLVVRGRIQRGETVLIHSGSGGVGQAAISIALSLGCRVFTTVGSAEKRAYLQARFPQLDDTSFANSRDTSFEQHVLLHTGGKGVDLVLNSLAEEKLQASVRCLAQHGRFLEIGKFDLSNNHPLGMAIFLKNVTFHGILLDALFEEANDSWREVAALLKAGIRDGVVKPLKCTVFPKAQVEDAFRYMAQGKHIGKVLVQVREEEPEAVLPGAQPTLISAISKTFCPAHKSYIITGGLGGFGLELARWLVLRGAQRLVLTSRSGIRTGYQAKHIREWRRQGIQVLVSTSNVSSLEGARALIAEATKLGPVGGVFNLAMVLRDAMLENQTPELFQDVNKPKYNGTLNLDRATREACPELDYFVAFSSVSCGRGNAGQTNYGFANSTMERICEQRRHDGLPGLAVQWGAIGDVGIVLEAMGTNDTVIGGTLPQRISSCMEVLDLFLNQPHAVLSSFVLAEKKAVAHGDGDTQRDLVKAVAHILGIRDLAGINLDSTLADLGLDSLMGVEVRQILEREHDLVLPMREVRQLTLRKLQEMSSKTDSATDTTAPKSRSDTSLKQNQAAAADTLLILGDSLSAGYRMSASAAWPALLNDKWQSKTSVVNASISGDTSQQGLARLPALLKQHQPRWVLVELGGNDGLRGFQPQQTEQTLRQILQDVKAANAEPLLMQIRLPANYGRRYNEAFSAIYPKLAKEFDVPLLPFFMEEVYLKPQWMQDDGIHPNRDAQPFIADWMAKQLQPLVNHDS

SEQ ID NO: 11 - protein, 2394 aa, synthetic construct
MEEVVIAGMSGKLPESENLQEFWANLIGGVDMVTDDDRRWKAGLYGLPKRSGKLKDLSKFDASFFGVHPKQAHTMDPQLRLLLEVSYEAIVDGGINPASLRGTNTGVWVGVSSSEASEALSRDPETLLGYSMVGCQRAMMANRLSFFFDFKGPSIALDTACSSSLLALQNAYQAIRSGECPAALVGGINLLLKPNTSVQFMKLGMLSPDGTCRSFDDSGSGYCRSEAVVAVLLTKKSLARRVYATILNAGTNTDGSKEQGVTFPSGEVQEQLICSLYQPAGLAPESLEYIEAHGTGTKVGDPQELNGITRSLCAFRQAPLLIGSTKSNMGHPEPASGLAALTKVLLSLEHGVWAPNLHFHNPNPEIPALLDGRLQVVDRPLPVRGGNVGINSFGFGGSNVHVILQPNTRQAPAPTAHAALPHLLHASGRTLEAVQDLLEQGRQHSQDLAFVSMLNDIAATPTAAMPFRGYTVLGVEGRVQEVQQVSTNKRPLWFICSGMGTQWRGMGLSLMRLDSFRESILRSDEAVKPLGVKVSDLLLSTDERTFDDIVHAFVSLTAIQIALIDLLTSVGLKPDGIIGHSLGEVACGYADGCLSQREAVLAAYWRGQCIKDAHLPPGSMAAVGLSWEECKQRCPAGVVPACHNSEDTVTISGPQAAVNEFVEQLKQEGVFAKEVRTGGLAFHSYFMEGIAPTLLQALKKVIREPRPRSARWLSTSIPEAQWQSSLARTSSAEYNVNNLVSPVLFQEALWHIPEHAVVLEIAPHALLQAVLKRGVKSSCTIIPLMKRDHKDNLEFFLTNLGKVHLTGINVNPNALFPPVEFPAPRGTPLISPHIKWDHSQTWDVPVAEDFPNGSSSSSATVYSIDASPESPDHYLVDHCIDGRVIFPGTGYLCLVWKTLARSLGLSLEETPVVFENVSFHQATILPKTGTVALEVRLLEASHAFEVSDTGNLIVSGKVYLWEDPNSKLFDHPEVPTPPESASVSRLTQGEVYKELRLRGYDYGPQFQGICEATLEGEQGKLLWKDNWVTFMDTMLQVSILGSSQQSLQLPTRVTAIYIDPATHRQKVYRLKEDTQVADVTTSRCLGITVSGGIHISRLQTTATSRRQQEQLVPTLEKFVFTPHMEAECLSESTALQKELQLCKGLARALQTKATQQGLKAAMLGQEDPPQHGLPRLLAAACQLQLNGNLQLELGEALAQERLLLPEDPLISGLLNSQALKACVDTALENLSTLKMKVAEVLAGEGHLYSRIPALLNTQPMLQLEYTATDRHPQALKDVQTKLQQHDVAQGQWNPSDPAPSSLGALDLLVCNCALATLGDPALALDNMVAALKEGGFLLVHTVLKGHALGETLACLPSEVQPAPSLLSQEEWESLFSRKALHLVGLKRSFYGTALFLCRRAIPQEKPIFLSVEDTSFQWVDSLKSTLATSSSQPVWLTAMDCPTSGVVGLVNCLRKEPGGHRIRCILLSNLSNTSHAPKLDPGSPELQQVLKHDLVMNVYRDGAWGAFRHFQLEQDKPKEQTAHAFVNVLTRGDLASIRWVSSPLKHTQPSSSGAQLCTVYYASLNFRDIMLATGKLSPDAIPGKWASRDCMLGMEFSGRDRCGRRVMGLVPAEGLATSVLLSSDFLWDVPSSWTLEEAASVPVVYTTAYYSLVVRGRIQRGETVLIHSGSGGVGQAAISIALSLGCRVFTTVGSAEKRAYLQARFPQLDDTSFANSRDTSFEQHVLLHTGGKGVDLVLNSLAEEKLQASVRCLAQHGRFLEIGKFDLSNNHPLGMAIFLKNVTFHGILLDALFEEANDSWREVAALLKAGIRDGVVKPLKCTVFPKAQVEDAFRYMAQGKHIGKVLVQVREEEPEAVLPGAQPTLISAISKTFCPAHKSYIITGGLGGFGLELARWLVLRGAQRLVLTSRSGIRTGYQAKHIREWRRQGIQVLVSTSNVSSLEGARALIAEATKLGPVGGVFNLAMVLRDAMLENQTPELFQDVNKPKYNGTLNLDRATREACPELDYFVAFSSVSCGRGNAGQTNYGFANSTMERICEQRRHDGLPGLAVQWGAIGDVGIVLEAMGTNDTVIGGTLPQRISSCMEVLDLFLNQPHAVLSSFVLAEKKAVAHGDGDTQRDLVKAVAHILGIRDLAGINLDSTLADLGLDSLMGVEVRQILEREHDLVLPMREVRQLTLRKLQEMSSKTDSATDTTAPKSRSDTSLKQNQAAAADTLLILGDSLSAGYRMSASAAWPALLNDKWQSKTSVVNASISGDTSQQGLARLPALLKQHQPRWVLVELGGNDGLRGFQPQQTEQTLRQILQDVKAANAEPLLMQIRPPANYGRRYNEAFSAIYPKLAKEFDVPLLPFFMEEVYLKPQWMQDDGIHPNRDAQPFIADWMAKQLQPLVNHDS

SEQ ID NO: 12 - protein, 2394 aa, synthetic construct
MEEVVIAGMSGKLPESENLQEFWANLIGGVDMVTDDDRRWKAGLYGLPKRSGKLKDLSKFDASFFGVHPKQAHTMDPQLRLLLEVSYEAIVDGGINPASLRGTNTGVWVGVSSSEASEALSRDPETLLGYSMVGCQRAMMANRLSFFFDFKGPSIALDTACSSSLLALQNAYQAIRSGECPAALVGGINLLLKPNTSVQFMKLGMLSPDGTCRSFDDSGSGYCRSEAVVAVLLTKKSLARRVYATILNAGTNTDGSKEQGVTFPSGEVQEQLICSLYQPAGLAPESLEYIEAHGTGTKVGDPQELNGITRSLCAFRQAPLLIGSTKSNMGHPEPASGLAALTKVLLSLEHGVWAPNLHFHNPNPEIPALLDGRLQVVDRPLPVRGGNVGINSFGFGGSNVHVILQPNTRQAPAPTAHAALPHLLHASGRTLEAVQDLLEQGRQHSQDLAFVSMLNDIAATPTAAMPFRGYTVLGVEGRVQEVQQVSTNKRPLWFICSGMGTQWRGMGLSLMRLDSFRESILRSDEAVKPLGVKVSDLLLSTDERTFDDIVHAFVSLTAIQIALIDLLTSVGLKPDGIIGHSLGEVACGYADGCLSQREAVLAAYWRGQCIKDAHLPPGSMAAVGLSWEECKQRCPAGVVPACHNSEDTVTISGPQAAVNEFVEQLKQEGVFAKEVRTGGLAFHSYFMEGIAPTLLQALKKVIREPRPRSARWLSTSIPEAQWQSSLARTSSAEYNVNNLVSPVLFQEALWHIPEHAVVLEIAPHALLQAVLKRGVKSSCTIIPLMKRDHKDNLEFFLTNLGKVHLTGINVNPNALFPPVEFPAPRGTPLISPHIKWDHSQTWDVPVAEDFPNGSSSSSATVYSIDASPESPDHYLVDHCIDGRVIFPGTGYLCLVWKTLARSLGLSLEETPVVFENVSFHQATILPKTGTVALEVRLLEASHAFEVSDTGNLIVSGKVYLWEDPNSKLFDHPEVPTPPESASVSRLTQGEVYKELRLRGYDYGPQFQGICEATLEGEQGKLLWKDNWVTFMDTMLQVSILGSSQQSLQLPTRVTAIYIDPATHRQKVYRLKEDTQVADVTTSRCLGITVSGGIHISRLQTTATSRRQQEQLVPTLEKFVFTPHMEAECLSESTALQKELQLCKGLARALQTKATQQGLKAAMLGQEDPPQHGLPRLLAAACQLQLNGNLQLELGEALAQERLLLPEDPLISGLLNSQALKACVDTALENLSTLKMKVAEVLAGEGHLYSRIPALLNTQPMLQLEYTATDRHPQALKDVQTKLQQHDVAQGQWNPSDPAPSSLGALDLLVCNCALATLGDPALALDNMVAALKEGGFLLVHTVLKGHALGETLACLPSEVQPAPSLLSQEEWESLFSRKALHLVGLKRSFYGTALFLCRRAIPQEKPIFLSVEDTSFQWVDSLKSTLATSSSQPVWLTAMDCPTSGVVGLVNCLRKEPGGHRIRCILLSNLSNTSHAPKLDPGSPELQQVLKHDLVMNVYRDGAWGAFRHFQLEQDKPKEQTAHAFVNVLTRGDLASIRWVSSPLKHTQPSSSGAQLCTVYYASLNFRDIMLATGKLSPDAIPGKWASRDCMLGMEFSGRDRCGRRVMGLVPAEGLATSVLLSSDFLWDVPSSWTLEEAASVPVVYTTAYYSLVVRGRIQRGETVLIHSGSGGVGQAAISIALSLGCRVFTTVGSAEKRAYLQARFPQLDDTSFANSRDTSFEQHVLLHTGGKGVDLVLNSLAEEKLQASVRCLAQHGRFLEIGKFDLSNNHPLGMAIFLKNVTFHGILLDALFEEANDSWREVAALLKAGIRDGVVKPLKCTVFPKAQVEDAFRYMAQGKHIGKVLVQVREEEPEAVLPGAQPTLISAISKTFCPAHKSYIITGGLGGFGLELARWLVLRGAQRLVLTSRSGIRTGYQAKHIREWRRQGIQVLVSTSNVSSLEGARALIAEATKLGPVGGVFNLAMVLRDAMLENQTPELFQDVNKPKYNGTLNLDRATREACPELDYFVAFSSVSCGRGNAGQTNYGFANSTMERICEQRRHDGLPGLAVQWGAIGDVGIVLEAMGTNDTVIGGTLPQRISSCMEVLDLFLNQPHAVLSSFVLAEKKAVAHGDGDTQRDLVKAVAHILGIRDLAGINLDSTLADLGLDSLMGVEVRQILEREHDLVLPMREVRQLTLRKLQEMSSKTDSATDTTAPKSRSDTSLKQNQAAAADTLLILGDSLSAGYRMSASAAWPALLNDKWQSKTSVVNASISGDTSQQGLARLPALLKQHQPRWVLVELGGNDGLRGFQPQQTEQTLRQILQDVKAANAEPLLMQIRLPANYGRRYNEAFSAIYPKLAKEFDVPLLPFFLDEVGKKPQWMQDDGIHPNRDAQPFIADWMAKQLQPLVNHDS

SEQ ID NO: 13 - protein, 2504 aa, synthetic construct
MEEVVIAGMSGKLPESENLQEFWANLIGGVDMVTDDDRRWKAGLYGLPKRSGKLKDLSKFDASFFGVHPKQAHTMDPQLRLLLEVSYEAIVDGGINPASLRGTNTGVWVGVSMSEASEALSRDPETLLGYSMVGCQRAMMANRLSFFFDFKGPSIALDTACSSSLLALQNAYQAIRSGECPAALVGGINLLLKPNTSVQFMKLGMLSPDGTCRSFDDSGSGYCRSEAVVAVLLTKKSLARRVYATILNAGTNTDGSKEQGVTFPSGEVQEQLICSLYQPAGLAPESLEYIEAHGTGTKVGDPQELNGITRSLCAFRQAPLLIGSTKSNMGHPEPASGLAALTKVLLSLEHGVWAPNLHFHNPNPEIPALLDGRLQVVDRPLPVRGGNVGINSFGFGGSNVHVILQPNTRQAPAPTAHAALPHLLHASGRTLEAVQDLLEQGRQHSQDLAFVSMLNDIAATPTAAMPFRGYTVLGVEGRVQEVQQVSTNKRPLWFICSGMGTQWRGMGLSLMRLDSFRESILRSDEAVKPLGVKVSDLLLSTDERTFDDIVHAFVSLTAIQIALIDLLTSVGLKPDGIIGHSLGEVACGYADGCLSQREAVLAAYWRGQCIKDAHLPPGSMAAVGLSWEECKQRCPAGVVPACHNSEDTVTISGPQAAVNEFVEQLKQEGVFAKEVRTGGLAFHSYFMEGIAPTLLQALKKVIREPRPRSARWLSTSIPEAQWQSSLARTSSAEYNVNNLVSPVLFQEALWHIPEHAVVLEIAPHALLQAVLKRGVKSSCTIIPLMKRDHKDNLEFFLTNLGKVHLTGINVNPNALFPPVEFPAPRGTPLISPHIKWDHSQTWDVPVAEDFPNGSSSSSATVYSIDASPESPDHYLVDHCIDGRVIFPGTGYLCLVWKTLARSLGLSLEETPVVFENVSFHQATILPKTGTVALEVRLLEASHAFEVSDTGNLIVSGKVYLWEDPNSKLFDHPEVPTPPESASVSRLTQGEVYKELRLRGYDYGPQFQGICEATLEGEQGKLLWKDNWVTFMDTMLQVSILGSSQQSLQLPTRVTAIYIDPATHRQKVYRLKEDTQVADVTTSRCLGITVSGGIHISRLQTTATSRRQQEQLVPTLEKFVFTPHMEAECLSESTALQKELQLCKGLARALQTKATQQGLKAAMLGQEDPPQHGLPRLLAAACQLQLNGNLQLELGEALAQERLLLPEDPLISGLLNSQALKACVDTALENLSTLKMKVAEVLAGEGHLYSRIPALLNTQPMLQLEYTATDRHPQALKDVQTKLQQHDVAQGQWNPSDPAPSSLGALDLLVCNCALATLGDPALALDNMVAALKEGGFLLVHTVLKGHALGETLACLPSEVQPAPSLLSQEEWESLFSRKALHLVGLKRSFYGTALFLCRRAIPQEKPIFLSVEDTSFQWVDSLKSTLATSSSQPVWLTAMDCPTSGVVGLVNCLRKEPGGHRIRCILLSNLSNTSHAPKLDPGSPELQQVLKHDLVMNVYRDGAWGAFRHFQLEQDKPKEQTAHAFVNVLTRGDLASIRWVSSPLKHTQPSSSGAQLCTVYYASLNFRDIMLATGKLSPDAIPGKWASRDCMLGMEFSGRDRCGRRVMGLVPAEGLATSVLLSSDFLWDVPSSWTLEEAASVPVVYTTAYYSLVVRGRIQRGETVLIHSGSGGVGQAAISIALSLGCRVFTTVGSAEKRAYLQARFPQLDDTSFANSRDTSFEQHVLLHTGGKGVDLVLNSLAEEKLQASVRCLAQHGRFLEIGKFDLSNNHPLGMAIFLKNVTFHGILLDALFEEANDSWREVAALLKAGIRDGVVKPLKCTVFPKAQVEDAFRYMAQGKHIGKVLVQVREEEPEAVLPGAQPTLISAISKTFCPAHKSYIITGGLGGFGLELARWLVLRGAQRLVLTSRSGIRTGYQAKHIREWRRQGIQVLVSTSNVSSLEGARALIAEATKLGPVGGVFNLAMVLRDAMLENQTPELFQDVNKPKYNGTLNLDRATREACPELDYFVAFSSVSCGRGNAGQTNYGFANSTMERICEQRRHDGLPGLAVQWGAIGDVGIVLEAMGTNDTVIGGTLPQRISSCMEVLDLFLNQPHAVLSSFVLAEKKAVAHGDGDTQRDLVKAVAHILGIRDLAGINLDSTLADLGLDSLMGVEVRQILEREHDLVLPMREVRQLTLRKLQEMSSKTDSATDTTAPKSRSDTSLKQNQLNLSTLLVNPEGPTLTQLNSVQSSERPLFLVHPIEGSTTVFHSLAAKLSVPTYGLQCTQAAPLDSIPNLAAYYIDCIKQVQPEGPYRIAGYSFGACVAFEMCSQLQAQQGPAPTHNNLFLFDGSHTYVLAYTQSYRAKMTPGCEAEAEAEALCFFIKQFLDVEHSKVLEALLPLKSLEDRVAASVDLITKSHHSLDRRELSFAAVSFYHKLRAADQYKPKAKYHGNVTLLRAKTGGTYGEDLGADYNLSQVCDGKVSVHIIEGDHRTLLEGSGLESIINIIHSSLAEPRVSVREG

SEQ ID NO: 14 - protein, 2394 aa, synthetic construct
MEEVVIAGMSGKLPESENLQEFWANLIGGVDMVTDDDRRWKAGLYGLPKRSGKLKDLSKFDASFFGVHPKQAHTMDPQLRLLLEVSYEAIVDGGINPASLRGTNTGVWVGVSMSEASEALSRDPETLLGYSMVGCQRAMMANRLSFFFDFKGPSIALDTACSSSLLALQNAYQAIRSGECPAALVGGINLLLKPNTSVQFMKLGMLSPDGTCRSFDDSGSGYCRSEAVVAVLLTKKSLARRVYATILNAGTNTDGSKEQGVTFPSGEVQEQLICSLYQPAGLAPESLEYIEAHGTGTKVGDPQELNGITRSLCAFRQAPLLIGSTKSNMGHPEPASGLAALTKVLLSLEHGVWAPNLHFHNPNPEIPALLDGRLQVVDRPLPVRGGNVGINSFGFGGSNVHVILQPNTRQAPAPTAHAALPHLLHASGRTLEAVQDLLEQGRQHSQDLAFVSMLNDIAATPTAAMPFRGYTVLGVEGRVQEVQQVSTNKRPLWFICSGMGTQWRGMGLSLMRLDSFRESILRSDEAVKPLGVKVSDLLLSTDERTFDDIVHAFVSLTAIQIALIDLLTSVGLKPDGIIGHSLGEVACGYADGCLSQREAVLAAYWRGQCIKDAHLPPGSMAAVGLSWEECKQRCPAGVVPACHNSEDTVTISGPQAAVNEFVEQLKQEGVFAKEVRTGGLAFHSYFMEGIAPTLLQALKKVIREPRPRSARWLSTSIPEAQWQSSLARTSSAEYNVNNLVSPVLFQEALWHIPEHAVVLEIAPHALLQAVLKRGVKSSCTIIPLMKRDHKDNLEFFLTNLGKVHLTGINVNPNALFPPVEFPAPRGTPLISPHIKWDHSQTWDVPVAEDFPNGSSSSSATVYSIDASPESPDHYLVDHCIDGRVIFPGTGYLCLVWKTLARSLGLSLEETPVVFENVSFHQATILPKTGTVALEVRLLEASHAFEVSDTGNLIVSGKVYLWEDPNSKLFDHPEVPTPPESASVSRLTQGEVYKELRLRGYDYGPQFQGICEATLEGEQGKLLWKDNWVTFMDTMLQVSILGSSQQSLQLPTRVTAIYIDPATHRQKVYRLKEDTQVADVTTSRCLGITVSGGIHISRLQTTATSRRQQEQLVPTLEKFVFTPHMEAECLSESTALQKELQLCKGLARALQTKATQQGLKAAMLGQEDPPQHGLPRLLAAACQLQLNGNLQLELGEALAQERLLLPEDPLISGLLNSQALKACVDTALENLSTLKMKVAEVLAGEGHLYSRIPALLNTQPMLQLEYTATDRHPQALKDVQTKLQQHDVAQGQWNPSDPAPSSLGALDLLVCNCALATLGDPALALDNMVAALKEGGFLLVHTVLKGHALGETLACLPSEVQPAPSLLSQEEWESLFSRKALHLVGLKRSFYGTALFLCRRAIPQEKPIFLSVEDTSFQWVDSLKSTLATSSSQPVWLTAMDCPTSGVVGLVNCLRKEPGGHRIRCILLSNLSNTSHAPKLDPGSPELQQVLKHDLVMNVYRDGAWGAFRHFQLEQDKPKEQTAHAFVNVLTRGDLASIRWVSSPLKHTQPSSSGAQLCTVYYASLNFRDIMLATGKLSPDAIPGKWASRDCMLGMEFSGRDRCGRRVMGLVPAEGLATSVLLSSDFLWDVPSSWTLEEAASVPVVYTTAYYSLVVRGRIQRGETVLIHSGSGGVGQAAISIALSLGCRVFTTVGSAEKRAYLQARFPQLDDTSFANSRDTSFEQHVLLHTGGKGVDLVLNSLAEEKLQASVRCLAQHGRFLEIGKFDLSNNHPLGMAIFLKNVTFHGILLDALFEEANDSWREVAALLKAGIRDGVVKPLKCTVFPKAQVEDAFRYMAQGKHIGKVLVQVREEEPEAVLPGAQPTLISAISKTFCPAHKSYIITGGLGGFGLELARWLVLRGAQRLVLTSRSGIRTGYQAKHIREWRRQGIQVLVSTSNVSSLEGARALIAEATKLGPVGGVFNLAMVLRDAMLENQTPELFQDVNKPKYNGTLNLDRATREACPELDYFVAFSSVSCGRGNAGQTNYGFANSTMERICEQRRHDGLPGLAVQWGAIGDVGIVLEAMGTNDTVIGGTLPQRISSCMEVLDLFLNQPHAVLSSFVLAEKKAVAHGDGDTQRDLVKAVAHILGIRDLAGINLDSTLADLGLDSLMGVEVRQILEREHDLVLPMREVRQLTLRKLQEMSSKTDSATDTTAPKSRSDTSLKQNQAAAADTLLILGDSLSAGYRMSASAAWPALLNDKWQSKTSVVNASISGDTSQQGLARLPALLKQHQPRWVLVELGGNDGLRGFQPQQTEQTLRQILQDVKAANAEPLLMQIRLPANYGRRYNEAFSAIYPKLAKEFDVPLLPFFMEEVYLKPQWMQDDGIHPNRDAQPFIADWMAKQLQPLVNHDS

SEQ ID NO: 15 - protein, 2394 aa, synthetic construct
MEEVVIAGMSGKLPESENLQEFWANLIGGVDMVTDDDRRWKAGLYGLPKRSGKLKDLSKFDASFFGVHPKQAHTMDPQLRLLLEVSYEAIVDGGINPASLRGTNTGVWVGVSMSEASEALSRDPETLLGYSMVGCQRAMMANRLSFFFDFKGPSIALDTACSSSLLALQNAYQAIRSGECPAALVGGINLLLKPNTSVQFMKLGMLSPDGTCRSFDDSGSGYCRSEAVVAVLLTKKSLARRVYATILNAGTNTDGSKEQGVTFPSGEVQEQLICSLYQPAGLAPESLEYIEAHGTGTKVGDPQELNGITRSLCAFRQAPLLIGSTKSNMGHPEPASGLAALTKVLLSLEHGVWAPNLHFHNPNPEIPALLDGRLQVVDRPLPVRGGNVGINSFGFGGSNVHVILQPNTRQAPAPTAHAALPHLLHASGRTLEAVQDLLEQGRQHSQDLAFVSMLNDIAATPTAAMPFRGYTVLGVEGRVQEVQQVSTNKRPLWFICSGMGTQWRGMGLSLMRLDSFRESILRSDEAVKPLGVKVSDLLLSTDERTFDDIVHAFVSLTAIQIALIDLLTSVGLKPDGIIGHSLGEVACGYADGCLSQREAVLAAYWRGQCIKDAHLPPGSMAAVGLSWEECKQRCPAGVVPACHNSEDTVTISGPQAAVNEFVEQLKQEGVFAKEVRTGGLAFHSYFMEGIAPTLLQALKKVIREPRPRSARWLSTSIPEAQWQSSLARTSSAEYNVNNLVSPVLFQEALWHIPEHAVVLEIAPHALLQAVLKRGVKSSCTIIPLMKRDHKDNLEFFLTNLGKVHLTGINVNPNALFPPVEFPAPRGTPLISPHIKWDHSQTWDVPVAEDFPNGSSSSSATVYSIDASPESPDHYLVDHCIDGRVIFPGTGYLCLVWKTLARSLGLSLEETPVVFENVSFHQATILPKTGTVALEVRLLEASHAFEVSDTGNLIVSGKVYLWEDPNSKLFDHPEVPTPPESASVSRLTQGEVYKELRLRGYDYGPQFQGICEATLEGEQGKLLWKDNWVTFMDTMLQVSILGSSQQSLQLPTRVTAIYIDPATHRQKVYRLKEDTQVADVTTSRCLGITVSGGIHISRLQTTATSRRQQEQLVPTLEKFVFTPHMEAECLSESTALQKELQLCKGLARALQTKATQQGLKAAMLGQEDPPQHGLPRLLAAACQLQLNGNLQLELGEALAQERLLLPEDPLISGLLNSQALKACVDTALENLSTLKMKVAEVLAGEGHLYSRIPALLNTQPMLQLEYTATDRHPQALKDVQTKLQQHDVAQGQWNPSDPAPSSLGALDLLVCNCALATLGDPALALDNMVAALKEGGFLLVHTVLKGHALGETLACLPSEVQPAPSLLSQEEWESLFSRKALHLVGLKRSFYGTALFLCRRAIPQEKPIFLSVEDTSFQWVDSLKSTLATSSSQPVWLTAMDCPTSGVVGLVNCLRKEPGGHRIRCILLSNLSNTSHAPKLDPGSPELQQVLKHDLVMNVYRDGAWGAFRHFQLEQDKPKEQTAHAFVNVLTRGDLASIRWVSSPLKHTQPSSSGAQLCTVYYASLNFRDIMLATGKLSPDAIPGKWASRDCMLGMEFSGRDRCGRRVMGLVPAEGLATSVLLSSDFLWDVPSSWTLEEAASVPVVYTTAYYSLVVRGRIQRGETVLIHSGSGGVGQAAISIALSLGCRVFTTVGSAEKRAYLQARFPQLDDTSFANSRDTSFEQHVLLHTGGKGVDLVLNSLAEEKLQASVRCLAQHGRFLEIGKFDLSNNHPLGMAIFLKNVTFHGILLDALFEEANDSWREVAALLKAGIRDGVVKPLKCTVFPKAQVEDAFRYMAQGKHIGKVLVQVREEEPEAVLPGAQPTLISAISKTFCPAHKSYIITGGLGGFGLELARWLVLRGAQRLVLTSRSGIRTGYQAKHIREWRRQGIQVLVSTSNVSSLEGARALIAEATKLGPVGGVFNLAMVLRDAMLENQTPELFQDVNKPKYNGTLNLDRATREACPELDYFVAFSSVSCGRGNAGQTNYGFANSTMERICEQRRHDGLPGLAVQWGAIGDVGIVLEAMGTNDTVIGGTLPQRISSCMEVLDLFLNQPHAVLSSFVLAEKKAVAHGDGDTQRDLVKAVAHILGIRDLAGINLDSTLADLGLDSLMGVEVRQILEREHDLVLPMREVRQLTLRKLQEMSSKTDSATDTTAPKSRSDTSLKQNQAAAADTLLILGDSLSAGYRMSASAAWPALLNDKWQSKTSVVNASISGDTSQQGLARLPALLKQHQPRWVLVELGGNDGLRGFQPQQTEQTLRQILQDVKAANAEPLLMQIRPPANYGRRYNEAFSAIYPKLAKEFDVPLLPFFMEEVYLKPQWMQDDGIHPNRDAQPFIADWMAKQLQPLVNHDS

SEQ ID NO: 16 - protein, 2394 aa, synthetic construct
MEEVVIAGMSGKLPESENLQEFWANLIGGVDMVTDDDRRWKAGLYGLPKRSGKLKDLSKFDASFFGVHPKQAHTMDPQLRLLLEVSYEAIVDGGINPASLRGTNTGVWVGVSMSEASEALSRDPETLLGYSMVGCQRAMMANRLSFFFDFKGPSIALDTACSSSLLALQNAYQAIRSGECPAALVGGINLLLKPNTSVQFMKLGMLSPDGTCRSFDDSGSGYCRSEAVVAVLLTKKSLARRVYATILNAGTNTDGSKEQGVTFPSGEVQEQLICSLYQPAGLAPESLEYIEAHGTGTKVGDPQELNGITRSLCAFRQAPLLIGSTKSNMGHPEPASGLAALTKVLLSLEHGVWAPNLHFHNPNPEIPALLDGRLQVVDRPLPVRGGNVGINSFGFGGSNVHVILQPNTRQAPAPTAHAALPHLLHASGRTLEAVQDLLEQGRQHSQDLAFVSMLNDIAATPTAAMPFRGYTVLGVEGRVQEVQQVSTNKRPLWFICSGMGTQWRGMGLSLMRLDSFRESILRSDEAVKPLGVKVSDLLLSTDERTFDDIVHAFVSLTAIQIALIDLLTSVGLKPDGIIGHSLGEVACGYADGCLSQREAVLAAYWRGQCIKDAHLPPGSMAAVGLSWEECKQRCPAGVVPACHNSEDTVTISGPQAAVNEFVEQLKQEGVFAKEVRTGGLAFHSYFMEGIAPTLLQALKKVIREPRPRSARWLSTSIPEAQWQSSLARTSSAEYNVNNLVSPVLFQEALWHIPEHAVVLEIAPHALLQAVLKRGVKSSCTIIPLMKRDHKDNLEFFLTNLGKVHLTGINVNPNALFPPVEFPAPRGTPLISPHIKWDHSQTWDVPVAEDFPNGSSSSSATVYSIDASPESPDHYLVDHCIDGRVIFPGTGYLCLVWKTLARSLGLSLEETPVVFENVSFHQATILPKTGTVALEVRLLEASHAFEVSDTGNLIVSGKVYLWEDPNSKLFDHPEVPTPPESASVSRLTQGEVYKELRLRGYDYGPQFQGICEATLEGEQGKLLWKDNWVTFMDTMLQVSILGSSQQSLQLPTRVTAIYIDPATHRQKVYRLKEDTQVADVTTSRCLGITVSGGIHISRLQTTATSRRQQEQLVPTLEKFVFTPHMEAECLSESTALQKELQLCKGLARALQTKATQQGLKAAMLGQEDPPQHGLPRLLAAACQLQLNGNLQLELGEALAQERLLLPEDPLISGLLNSQALKACVDTALENLSTLKMKVAEVLAGEGHLYSRIPALLNTQPMLQLEYTATDRHPQALKDVQTKLQQHDVAQGQWNPSDPAPSSLGALDLLVCNCALATLGDPALALDNMVAALKEGGFLLVHTVLKGHALGETLACLPSEVQPAPSLLSQEEWESLFSRKALHLVGLKRSFYGTALFLCRRAIPQEKPIFLSVEDTSFQWVDSLKSTLATSSSQPVWLTAMDCPTSGVVGLVNCLRKEPGGHRIRCILLSNLSNTSHAPKLDPGSPELQQVLKHDLVMNVYRDGAWGAFRHFQLEQDKPKEQTAHAFVNVLTRGDLASIRWVSSPLKHTQPSSSGAQLCTVYYASLNFRDIMLATGKLSPDAIPGKWASRDCMLGMEFSGRDRCGRRVMGLVPAEGLATSVLLSSDFLWDVPSSWTLEEAASVPVVYTTAYYSLVVRGRIQRGETVLIHSGSGGVGQAAISIALSLGCRVFTTVGSAEKRAYLQARFPQLDDTSFANSRDTSFEQHVLLHTGGKGVDLVLNSLAEEKLQASVRCLAQHGRFLEIGKFDLSNNHPLGMAIFLKNVTFHGILLDALFEEANDSWREVAALLKAGIRDGVVKPLKCTVFPKAQVEDAFRYMAQGKHIGKVLVQVREEEPEAVLPGAQPTLISAISKTFCPAHKSYIITGGLGGFGLELARWLVLRGAQRLVLTSRSGIRTGYQAKHIREWRRQGIQVLVSTSNVSSLEGARALIAEATKLGPVGGVFNLAMVLRDAMLENQTPELFQDVNKPKYNGTLNLDRATREACPELDYFVAFSSVSCGRGNAGQTNYGFANSTMERICEQRRHDGLPGLAVQWGAIGDVGIVLEAMGTNDTVIGGTLPQRISSCMEVLDLFLNQPHAVLSSFVLAEKKAVAHGDGDTQRDLVKAVAHILGIRDLAGINLDSTLADLGLDSLMGVEVRQILEREHDLVLPMREVRQLTLRKLQEMSSKTDSATDTTAPKSRSDTSLKQNQAAAADTLLILGDSLSAGYRMSASAAWPALLNDKWQSKTSVVNASISGDTSQQGLARLPALLKQHQPRWVLVELGGNDGLRGFQPQQTEQTLRQILQDVKAANAEPLLMQIRLPANYGRRYNEAFSAIYPKLAKEFDVPLLPFFLDEVGKKPQWMQDDGIHPNRDAQPFIADWMAKQLQPLVNHDS

SEQ ID NO: 17 - protein, 2504 aa, synthetic construct
MEEVVIAGMSGKLPESENLQEFWANLIGGVDMVTDDDRRWKAGLYGLPKRSGKLKDLSKFDASFFGVHPKQAHTMDPQLRLLLEVSYEAIVDGGINPASLRGTNTGVWVGVSFSEASEALSRDPETLLGYSMVGCQRAMMANRLSFFFDFKGPSIALDTACSSSLLALQNAYQAIRSGECPAALVGGINLLLKPNTSVQFMKLGMLSPDGTCRSFDDSGSGYCRSEAVVAVLLTKKSLARRVYATILNAGTNTDGSKEQGVTFPSGEVQEQLICSLYQPAGLAPESLEYIEAHGTGTKVGDPQELNGITRSLCAFRQAPLLIGSTKSNMGHPEPASGLAALTKVLLSLEHGVWAPNLHFHNPNPEIPALLDGRLQVVDRPLPVRGGNVGINSFGFGGSNVHVILQPNTRQAPAPTAHAALPHLLHASGRTLEAVQDLLEQGRQHSQDLAFVSMLNDIAATPTAAMPFRGYTVLGVEGRVQEVQQVSTNKRPLWFICSGMGTQWRGMGLSLMRLDSFRESILRSDEAVKPLGVKVSDLLLSTDERTFDDIVHAFVSLTAIQIALIDLLTSVGLKPDGIIGHSLGEVACGYADGCLSQREAVLAAYWRGQCIKDAHLPPGSMAAVGLSWEECKQRCPAGVVPACHNSEDTVTISGPQAAVNEFVEQLKQEGVFAKEVRTGGLAFHSYFMEGIAPTLLQALKKVIREPRPRSARWLSTSIPEAQWQSSLARTSSAEYNVNNLVSPVLFQEALWHIPEHAVVLEIAPHALLQAVLKRGVKSSCTIIPLMKRDHKDNLEFFLTNLGKVHLTGINVNPNALFPPVEFPAPRGTPLISPHIKWDHSQTWDVPVAEDFPNGSSSSSATVYSIDASPESPDHYLVDHCIDGRVIFPGTGYLCLVWKTLARSLGLSLEETPVVFENVSFHQATILPKTGTVALEVRLLEASHAFEVSDTGNLIVSGKVYLWEDPNSKLFDHPEVPTPPESASVSRLTQGEVYKELRLRGYDYGPQFQGICEATLEGEQGKLLWKDNWVTFMDTMLQVSILGSSQQSLQLPTRVTAIYIDPATHRQKVYRLKEDTQVADVTTSRCLGITVSGGIHISRLQTTATSRRQQEQLVPTLEKFVFTPHMEAECLSESTALQKELQLCKGLARALQTKATQQGLKAAMLGQEDPPQHGLPRLLAAACQLQLNGNLQLELGEALAQERLLLPEDPLISGLLNSQALKACVDTALENLSTLKMKVAEVLAGEGHLYSRIPALLNTQPMLQLEYTATDRHPQALKDVQTKLQQHDVAQGQWNPSDPAPSSLGALDLLVCNCALATLGDPALALDNMVAALKEGGFLLVHTVLKGHALGETLACLPSEVQPAPSLLSQEEWESLFSRKALHLVGLKRSFYGTALFLCRRAIPQEKPIFLSVEDTSFQWVDSLKSTLATSSSQPVWLTAMDCPTSGVVGLVNCLRKEPGGHRIRCILLSNLSNTSHAPKLDPGSPELQQVLKHDLVMNVYRDGAWGAFRHFQLEQDKPKEQTAHAFVNVLTRGDLASIRWVSSPLKHTQPSSSGAQLCTVYYASLNFRDIMLATGKLSPDAIPGKWASRDCMLGMEFSGRDRCGRRVMGLVPAEGLATSVLLSSDFLWDVPSSWTLEEAASVPVVYTTAYYSLVVRGRIQRGETVLIHSGSGGVGQAAISIALSLGCRVFTTVGSAEKRAYLQARFPQLDDTSFANSRDTSFEQHVLLHTGGKGVDLVLNSLAEEKLQASVRCLAQHGRFLEIGKFDLSNNHPLGMAIFLKNVTFHGILLDALFEEANDSWREVAALLKAGIRDGVVKPLKCTVFPKAQVEDAFRYMAQGKHIGKVLVQVREEEPEAVLPGAQPTLISAISKTFCPAHKSYIITGGLGGFGLELARWLVLRGAQRLVLTSRSGIRTGYQAKHIREWRRQGIQVLVSTSNVSSLEGARALIAEATKLGPVGGVFNLAMVLRDAMLENQTPELFQDVNKPKYNGTLNLDRATREACPELDYFVAFSSVSCGRGNAGQTNYGFANSTMERICEQRRHDGLPGLAVQWGAIGDVGIVLEAMGTNDTVIGGTLPQRISSCMEVLDLFLNQPHAVLSSFVLAEKKAVAHGDGDTQRDLVKAVAHILGIRDLAGINLDSTLADLGLDSLMGVEVRQILEREHDLVLPMREVRQLTLRKLQEMSSKTDSATDTTAPKSRSDTSLKQNQLNLSTLLVNPEGPTLTQLNSVQSSERPLFLVHPIEGSTTVFHSLAAKLSVPTYGLQCTQAAPLDSIPNLAAYYIDCIKQVQPEGPYRIAGYSFGACVAFEMCSQLQAQQGPAPTHNNLFLFDGSHTYVLAYTQSYRAKMTPGCEAEAEAEALCFFIKQFLDVEHSKVLEALLPLKSLEDRVAASVDLITKSHHSLDRRELSFAAVSFYHKLRAADQYKPKAKYHGNVTLLRAKTGGTYGEDLGADYNLSQVCDGKVSVHIIEGDHRTLLEGSGLESIINIIHSSLAEPRVSVREG

SEQ ID NO: 18 - protein, 2394 aa, synthetic construct
MEEVVIAGMSGKLPESENLQEFWANLIGGVDMVTDDDRRWKAGLYGLPKRSGKLKDLSKFDASFFGVHPKQAHTMDPQLRLLLEVSYEAIVDGGINPASLRGTNTGVWVGVSFSEASEALSRDPETLLGYSMVGCQRAMMANRLSFFFDFKGPSIALDTACSSSLLALQNAYQAIRSGECPAALVGGINLLLKPNTSVQFMKLGMLSPDGTCRSFDDSGSGYCRSEAVVAVLLTKKSLARRVYATILNAGTNTDGSKEQGVTFPSGEVQEQLICSLYQPAGLAPESLEYIEAHGTGTKVGDPQELNGITRSLCAFRQAPLLIGSTKSNMGHPEPASGLAALTKVLLSLEHGVWAPNLHFHNPNPEIPALLDGRLQVVDRPLPVRGGNVGINSFGFGGSNVHVILQPNTRQAPAPTAHAALPHLLHASGRTLEAVQDLLEQGRQHSQDLAFVSMLNDIAATPTAAMPFRGYTVLGVEGRVQEVQQVSTNKRPLWFICSGMGTQWRGMGLSLMRLDSFRESILRSDEAVKPLGVKVSDLLLSTDERTFDDIVHAFVSLTAIQIALIDLLTSVGLKPDGIIGHSLGEVACGYADGCLSQREAVLAAYWRGQCIKDAHLPPGSMAAVGLSWEECKQRCPAGVVPACHNSEDTVTISGPQAAVNEFVEQLKQEGVFAKEVRTGGLAFHSYFMEGIAPTLLQALKKVIREPRPRSARWLSTSIPEAQWQSSLARTSSAEYNVNNLVSPVLFQEALWHIPEHAVVLEIAPHALLQAVLKRGVKSSCTIIPLMKRDHKDNLEFFLTNLGKVHLTGINVNPNALFPPVEFPAPRGTPLISPHIKWDHSQTWDVPVAEDFPNGSSSSSATVYSIDASPESPDHYLVDHCIDGRVIFPGTGYLCLVWKTLARSLGLSLEETPVVFENVSFHQATILPKTGTVALEVRLLEASHAFEVSDTGNLIVSGKVYLWEDPNSKLFDHPEVPTPPESASVSRLTQGEVYKELRLRGYDYGPQFQGICEATLEGEQGKLLWKDNWVTFMDTMLQVSILGSSQQSLQLPTRVTAIYIDPATHRQKVYRLKEDTQVADVTTSRCLGITVSGGIHISRLQTTATSRRQQEQLVPTLEKFVFTPHMEAECLSESTALQKELQLCKGLARALQTKATQQGLKAAMLGQEDPPQHGLPRLLAAACQLQLNGNLQLELGEALAQERLLLPEDPLISGLLNSQALKACVDTALENLSTLKMKVAEVLAGEGHLYSRIPALLNTQPMLQLEYTATDRHPQALKDVQTKLQQHDVAQGQWNPSDPAPSSLGALDLLVCNCALATLGDPALALDNMVAALKEGGFLLVHTVLKGHALGETLACLPSEVQPAPSLLSQEEWESLFSRKALHLVGLKRSFYGTALFLCRRAIPQEKPIFLSVEDTSFQWVDSLKSTLATSSSQPVWLTAMDCPTSGVVGLVNCLRKEPGGHRIRCILLSNLSNTSHAPKLDPGSPELQQVLKHDLVMNVYRDGAWGAFRHFQLEQDKPKEQTAHAFVNVLTRGDLASIRWVSSPLKHTQPSSSGAQLCTVYYASLNFRDIMLATGKLSPDAIPGKWASRDCMLGMEFSGRDRCGRRVMGLVPAEGLATSVLLSSDFLWDVPSSWTLEEAASVPVVYTTAYYSLVVRGRIQRGETVLIHSGSGGVGQAAISIALSLGCRVFTTVGSAEKRAYLQARFPQLDDTSFANSRDTSFEQHVLLHTGGKGVDLVLNSLAEEKLQASVRCLAQHGRFLEIGKFDLSNNHPLGMAIFLKNVTFHGILLDALFEEANDSWREVAALLKAGIRDGVVKPLKCTVFPKAQVEDAFRYMAQGKHIGKVLVQVREEEPEAVLPGAQPTLISAISKTFCPAHKSYIITGGLGGFGLELARWLVLRGAQRLVLTSRSGIRTGYQAKHIREWRRQGIQVLVSTSNVSSLEGARALIAEATKLGPVGGVFNLAMVLRDAMLENQTPELFQDVNKPKYNGTLNLDRATREACPELDYFVAFSSVSCGRGNAGQTNYGFANSTMERICEQRRHDGLPGLAVQWGAIGDVGIVLEAMGTNDTVIGGTLPQRISSCMEVLDLFLNQPHAVLSSFVLAEKKAVAHGDGDTQRDLVKAVAHILGIRDLAGINLDSTLADLGLDSLMGVEVRQILEREHDLVLPMREVRQLTLRKLQEMSSKTDSATDTTAPKSRSDTSLKQNQAAAADTLLILGDSLSAGYRMSASAAWPALLNDKWQSKTSVVNASISGDTSQQGLARLPALLKQHQPRWVLVELGGNDGLRGFQPQQTEQTLRQILQDVKAANAEPLLMQIRLPANYGRRYNEAFSAIYPKLAKEFDVPLLPFFMEEVYLKPQWMQDDGIHPNRDAQPFIADWMAKQLQPLVNHDS

SEQ ID NO: 19 - protein, 2394 aa, synthetic construct
MEEVVIAGMSGKLPESENLQEFWANLIGGVDMVTDDDRRWKAGLYGLPKRSGKLKDLSKFDASFFGVHPKQAHTMDPQLRLLLEVSYEAIVDGGINPASLRGTNTGVWVGVSFSEASEALSRDPETLLGYSMVGCQRAMMANRLSFFFDFKGPSIALDTACSSSLLALQNAYQAIRSGECPAALVGGINLLLKPNTSVQFMKLGMLSPDGTCRSFDDSGSGYCRSEAVVAVLLTKKSLARRVYATILNAGTNTDGSKEQGVTFPSGEVQEQLICSLYQPAGLAPESLEYIEAHGTGTKVGDPQELNGITRSLCAFRQAPLLIGSTKSNMGHPEPASGLAALTKVLLSLEHGVWAPNLHFHNPNPEIPALLDGRLQVVDRPLPVRGGNVGINSFGFGGSNVHVILQPNTRQAPAPTAHAALPHLLHASGRTLEAVQDLLEQGRQHSQDLAFVSMLNDIAATPTAAMPFRGYTVLGVEGRVQEVQQVSTNKRPLWFICSGMGTQWRGMGLSLMRLDSFRESILRSDEAVKPLGVKVSDLLLSTDERTFDDIVHAFVSLTAIQIALIDLLTSVGLKPDGIIGHSLGEVACGYADGCLSQREAVLAAYWRGQCIKDAHLPPGSMAAVGLSWEECKQRCPAGVVPACHNSEDTVTISGPQAAVNEFVEQLKQEGVFAKEVRTGGLAFHSYFMEGIAPTLLQALKKVIREPRPRSARWLSTSIPEAQWQSSLARTSSAEYNVNNLVSPVLFQEALWHIPEHAVVLEIAPHALLQAVLKRGVKSSCTIIPLMKRDHKDNLEFFLTNLGKVHLTGINVNPNALFPPVEFPAPRGTPLISPHIKWDHSQTWDVPVAEDFPNGSSSSSATVYSIDASPESPDHYLVDHCIDGRVIFPGTGYLCLVWKTLARSLGLSLEETPVVFENVSFHQATILPKTGTVALEVRLLEASHAFEVSDTGNLIVSGKVYLWEDPNSKLFDHPEVPTPPESASVSRLTQGEVYKELRLRGYDYGPQFQGICEATLEGEQGKLLWKDNWVTFMDTMLQVSILGSSQQSLQLPTRVTAIYIDPATHRQKVYRLKEDTQVADVTTSRCLGITVSGGIHISRLQTTATSRRQQEQLVPTLEKFVFTPHMEAECLSESTALQKELQLCKGLARALQTKATQQGLKAAMLGQEDPPQHGLPRLLAAACQLQLNGNLQLELGEALAQERLLLPEDPLISGLLNSQALKACVDTALENLSTLKMKVAEVLAGEGHLYSRIPALLNTQPMLQLEYTATDRHPQALKDVQTKLQQHDVAQGQWNPSDPAPSSLGALDLLVCNCALATLGDPALALDNMVAALKEGGFLLVHTVLKGHALGETLACLPSEVQPAPSLLSQEEWESLFSRKALHLVGLKRSFYGTALFLCRRAIPQEKPIFLSVEDTSFQWVDSLKSTLATSSSQPVWLTAMDCPTSGVVGLVNCLRKEPGGHRIRCILLSNLSNTSHAPKLDPGSPELQQVLKHDLVMNVYRDGAWGAFRHFQLEQDKPKEQTAHAFVNVLTRGDLASIRWVSSPLKHTQPSSSGAQLCTVYYASLNFRDIMLATGKLSPDAIPGKWASRDCMLGMEFSGRDRCGRRVMGLVPAEGLATSVLLSSDFLWDVPSSWTLEEAASVPVVYTTAYYSLVVRGRIQRGETVLIHSGSGGVGQAAISIALSLGCRVFTTVGSAEKRAYLQARFPQLDDTSFANSRDTSFEQHVLLHTGGKGVDLVLNSLAEEKLQASVRCLAQHGRFLEIGKFDLSNNHPLGMAIFLKNVTFHGILLDALFEEANDSWREVAALLKAGIRDGVVKPLKCTVFPKAQVEDAFRYMAQGKHIGKVLVQVREEEPEAVLPGAQPTLISAISKTFCPAHKSYIITGGLGGFGLELARWLVLRGAQRLVLTSRSGIRTGYQAKHIREWRRQGIQVLVSTSNVSSLEGARALIAEATKLGPVGGVFNLAMVLRDAMLENQTPELFQDVNKPKYNGTLNLDRATREACPELDYFVAFSSVSCGRGNAGQTNYGFANSTMERICEQRRHDGLPGLAVQWGAIGDVGIVLEAMGTNDTVIGGTLPQRISSCMEVLDLFLNQPHAVLSSFVLAEKKAVAHGDGDTQRDLVKAVAHILGIRDLAGINLDSTLADLGLDSLMGVEVRQILEREHDLVLPMREVRQLTLRKLQEMSSKTDSATDTTAPKSRSDTSLKQNQAAAADTLLILGDSLSAGYRMSASAAWPALLNDKWQSKTSVVNASISGDTSQQGLARLPALLKQHQPRWVLVELGGNDGLRGFQPQQTEQTLRQILQDVKAANAEPLLMQIRPPANYGRRYNEAFSAIYPKLAKEFDVPLLPFFMEEVYLKPQWMQDDGIHPNRDAQPFIADWMAKQLQPLVNHDS

SEQ ID NO: 20 - protein, 2394 aa, synthetic construct
MEEVVIAGMSGKLPESENLQEFWANLIGGVDMVTDDDRRWKAGLYGLPKRSGKLKDLSKFDASFFGVHPKQAHTMDPQLRLLLEVSYEAIVDGGINPASLRGTNTGVWVGVSFSEASEALSRDPETLLGYSMVGCQRAMMANRLSFFFDFKGPSIALDTACSSSLLALQNAYQAIRSGECPAALVGGINLLLKPNTSVQFMKLGMLSPDGTCRSFDDSGSGYCRSEAVVAVLLTKKSLARRVYATILNAGTNTDGSKEQGVTFPSGEVQEQLICSLYQPAGLAPESLEYIEAHGTGTKVGDPQELNGITRSLCAFRQAPLLIGSTKSNMGHPEPASGLAALTKVLLSLEHGVWAPNLHFHNPNPEIPALLDGRLQVVDRPLPVRGGNVGINSFGFGGSNVHVILQPNTRQAPAPTAHAALPHLLHASGRTLEAVQDLLEQGRQHSQDLAFVSMLNDIAATPTAAMPFRGYTVLGVEGRVQEVQQVSTNKRPLWFICSGMGTQWRGMGLSLMRLDSFRESILRSDEAVKPLGVKVSDLLLSTDERTFDDIVHAFVSLTAIQIALIDLLTSVGLKPDGIIGHSLGEVACGYADGCLSQREAVLAAYWRGQCIKDAHLPPGSMAAVGLSWEECKQRCPAGVVPACHNSEDTVTISGPQAAVNEFVEQLKQEGVFAKEVRTGGLAFHSYFMEGIAPTLLQALKKVIREPRPRSARWLSTSIPEAQWQSSLARTSSAEYNVNNLVSPVLFQEALWHIPEHAVVLEIAPHALLQAVLKRGVKSSCTIIPLMKRDHKDNLEFFLTNLGKVHLTGINVNPNALFPPVEFPAPRGTPLISPHIKWDHSQTWDVPVAEDFPNGSSSSSATVYSIDASPESPDHYLVDHCIDGRVIFPGTGYLCLVWKTLARSLGLSLEETPVVFENVSFHQATILPKTGTVALEVRLLEASHAFEVSDTGNLIVSGKVYLWEDPNSKLFDHPEVPTPPESASVSRLTQGEVYKELRLRGYDYGPQFQGICEATLEGEQGKLLWKDNWVTFMDTMLQVSILGSSQQSLQLPTRVTAIYIDPATHRQKVYRLKEDTQVADVTTSRCLGITVSGGIHISRLQTTATSRRQQEQLVPTLEKFVFTPHMEAECLSESTALQKELQLCKGLARALQTKATQQGLKAAMLGQEDPPQHGLPRLLAAACQLQLNGNLQLELGEALAQERLLLPEDPLISGLLNSQALKACVDTALENLSTLKMKVAEVLAGEGHLYSRIPALLNTQPMLQLEYTATDRHPQALKDVQTKLQQHDVAQGQWNPSDPAPSSLGALDLLVCNCALATLGDPALALDNMVAALKEGGFLLVHTVLKGHALGETLACLPSEVQPAPSLLSQEEWESLFSRKALHLVGLKRSFYGTALFLCRRAIPQEKPIFLSVEDTSFQWVDSLKSTLATSSSQPVWLTAMDCPTSGVVGLVNCLRKEPGGHRIRCILLSNLSNTSHAPKLDPGSPELQQVLKHDLVMNVYRDGAWGAFRHFQLEQDKPKEQTAHAFVNVLTRGDLASIRWVSSPLKHTQPSSSGAQLCTVYYASLNFRDIMLATGKLSPDAIPGKWASRDCMLGMEFSGRDRCGRRVMGLVPAEGLATSVLLSSDFLWDVPSSWTLEEAASVPVVYTTAYYSLVVRGRIQRGETVLIHSGSGGVGQAAISIALSLGCRVFTTVGSAEKRAYLQARFPQLDDTSFANSRDTSFEQHVLLHTGGKGVDLVLNSLAEEKLQASVRCLAQHGRFLEIGKFDLSNNHPLGMAIFLKNVTFHGILLDALFEEANDSWREVAALLKAGIRDGVVKPLKCTVFPKAQVEDAFRYMAQGKHIGKVLVQVREEEPEAVLPGAQPTLISAISKTFCPAHKSYIITGGLGGFGLELARWLVLRGAQRLVLTSRSGIRTGYQAKHIREWRRQGIQVLVSTSNVSSLEGARALIAEATKLGPVGGVFNLAMVLRDAMLENQTPELFQDVNKPKYNGTLNLDRATREACPELDYFVAFSSVSCGRGNAGQTNYGFANSTMERICEQRRHDGLPGLAVQWGAIGDVGIVLEAMGTNDTVIGGTLPQRISSCMEVLDLFLNQPHAVLSSFVLAEKKAVAHGDGDTQRDLVKAVAHILGIRDLAGINLDSTLADLGLDSLMGVEVRQILEREHDLVLPMREVRQLTLRKLQEMSSKTDSATDTTAPKSRSDTSLKQNQAAAADTLLILGDSLSAGYRMSASAAWPALLNDKWQSKTSVVNASISGDTSQQGLARLPALLKQHQPRWVLVELGGNDGLRGFQPQQTEQTLRQILQDVKAANAEPLLMQIRLPANYGRRYNEAFSAIYPKLAKEFDVPLLPFFLDEVGKKPQWMQDDGIHPNRDAQPFIADWMAKQLQPLVNHDS

SEQ ID NO: 21 - protein, 2504 aa, synthetic construct
MEEVVIAGMSGKLPESENLQEFWANLIGGVDMVTDDDRRWKAGLYGLPKRSGKLKDLSKFDASFFGVHPKQAHTMDPQLRLLLEVSYEAIVDGGINPASLRGTNTGVWVGVSWSEASEALSRDPETLLGYSMVGCQRAMMANRLSFFFDFKGPSIALDTACSSSLLALQNAYQAIRSGECPAALVGGINLLLKPNTSVQFMKLGMLSPDGTCRSFDDSGSGYCRSEAVVAVLLTKKSLARRVYATILNAGTNTDGSKEQGVTFPSGEVQEQLICSLYQPAGLAPESLEYIEAHGTGTKVGDPQELNGITRSLCAFRQAPLLIGSTKSNMGHPEPASGLAALTKVLLSLEHGVWAPNLHFHNPNPEIPALLDGRLQVVDRPLPVRGGNVGINSFGFGGSNVHVILQPNTRQAPAPTAHAALPHLLHASGRTLEAVQDLLEQGRQHSQDLAFVSMLNDIAATPTAAMPFRGYTVLGVEGRVQEVQQVSTNKRPLWFICSGMGTQWRGMGLSLMRLDSFRESILRSDEAVKPLGVKVSDLLLSTDERTFDDIVHAFVSLTAIQIALIDLLTSVGLKPDGIIGHSLGEVACGYADGCLSQREAVLAAYWRGQCIKDAHLPPGSMAAVGLSWEECKQRCPAGVVPACHNSEDTVTISGPQAAVNEFVEQLKQEGVFAKEVRTGGLAFHSYFMEGIAPTLLQALKKVIREPRPRSARWLSTSIPEAQWQSSLARTSSAEYNVNNLVSPVLFQEALWHIPEHAVVLEIAPHALLQAVLKRGVKSSCTIIPLMKRDHKDNLEFFLTNLGKVHLTGINVNPNALFPPVEFPAPRGTPLISPHIKWDHSQTWDVPVAEDFPNGSSSSSATVYSIDASPESPDHYLVDHCIDGRVIFPGTGYLCLVWKTLARSLGLSLEETPVVFENVSFHQATILPKTGTVALEVRLLEASHAFEVSDTGNLIVSGKVYLWEDPNSKLFDHPEVPTPPESASVSRLTQGEVYKELRLRGYDYGPQFQGICEATLEGEQGKLLWKDNWVTFMDTMLQVSILGSSQQSLQLPTRVTAIYIDPATHRQKVYRLKEDTQVADVTTSRCLGITVSGGIHISRLQTTATSRRQQEQLVPTLEKFVFTPHMEAECLSESTALQKELQLCKGLARALQTKATQQGLKAAMLGQEDPPQHGLPRLLAAACQLQLNGNLQLELGEALAQERLLLPEDPLISGLLNSQALKACVDTALENLSTLKMKVAEVLAGEGHLYSRIPALLNTQPMLQLEYTATDRHPQALKDVQTKLQQHDVAQGQWNPSDPAPSSLGALDLLVCNCALATLGDPALALDNMVAALKEGGFLLVHTVLKGHALGETLACLPSEVQPAPSLLSQEEWESLFSRKALHLVGLKRSFYGTALFLCRRAIPQEKPIFLSVEDTSFQWVDSLKSTLATSSSQPVWLTAMDCPTSGVVGLVNCLRKEPGGHRIRCILLSNLSNTSHAPKLDPGSPELQQVLKHDLVMNVYRDGAWGAFRHFQLEQDKPKEQTAHAFVNVLTRGDLASIRWVSSPLKHTQPSSSGAQLCTVYYASLNFRDIMLATGKLSPDAIPGKWASRDCMLGMEFSGRDRCGRRVMGLVPAEGLATSVLLSSDFLWDVPSSWTLEEAASVPVVYTTAYYSLVVRGRIQRGETVLIHSGSGGVGQAAISIALSLGCRVFTTVGSAEKRAYLQARFPQLDDTSFANSRDTSFEQHVLLHTGGKGVDLVLNSLAEEKLQASVRCLAQHGRFLEIGKFDLSNNHPLGMAIFLKNVTFHGILLDALFEEANDSWREVAALLKAGIRDGVVKPLKCTVFPKAQVEDAFRYMAQGKHIGKVLVQVREEEPEAVLPGAQPTLISAISKTFCPAHKSYIITGGLGGFGLELARWLVLRGAQRLVLTSRSGIRTGYQAKHIREWRRQGIQVLVSTSNVSSLEGARALIAEATKLGPVGGVFNLAMVLRDAMLENQTPELFQDVNKPKYNGTLNLDRATREACPELDYFVAFSSVSCGRGNAGQTNYGFANSTMERICEQRRHDGLPGLAVQWGAIGDVGIVLEAMGTNDTVIGGTLPQRISSCMEVLDLFLNQPHAVLSSFVLAEKKAVAHGDGDTQRDLVKAVAHILGIRDLAGINLDSTLADLGLDSLMGVEVRQILEREHDLVLPMREVRQLTLRKLQEMSSKTDSATDTTAPKSRSDTSLKQNQLNLSTLLVNPEGPTLTQLNSVQSSERPLFLVHPIEGSTTVFHSLAAKLSVPTYGLQCTQAAPLDSIPNLAAYYIDCIKQVQPEGPYRIAGYSFGACVAFEMCSQLQAQQGPAPTHNNLFLFDGSHTYVLAYTQSYRAKMTPGCEAEAEAEALCFFIKQFLDVEHSKVLEALLPLKSLEDRVAASVDLITKSHHSLDRRELSFAAVSFYHKLRAADQYKPKAKYHGNVTLLRAKTGGTYGEDLGADYNLSQVCDGKVSVHIIEGDHRTLLEGSGLESIINIIHSSLAEPRVSVREG

SEQ ID NO: 22 - protein, 2394 aa, synthetic construct
MEEVVIAGMSGKLPESENLQEFWANLIGGVDMVTDDDRRWKAGLYGLPKRSGKLKDLSKFDASFFGVHPKQAHTMDPQLRLLLEVSYEAIVDGGINPASLRGTNTGVWVGVSWSEASEALSRDPETLLGYSMVGCQRAMMANRLSFFFDFKGPSIALDTACSSSLLALQNAYQAIRSGECPAALVGGINLLLKPNTSVQFMKLGMLSPDGTCRSFDDSGSGYCRSEAVVAVLLTKKSLARRVYATILNAGTNTDGSKEQGVTFPSGEVQEQLICSLYQPAGLAPESLEYIEAHGTGTKVGDPQELNGITRSLCAFRQAPLLIGSTKSNMGHPEPASGLAALTKVLLSLEHGVWAPNLHFHNPNPEIPALLDGRLQVVDRPLPVRGGNVGINSFGFGGSNVHVILQPNTRQAPAPTAHAALPHLLHASGRTLEAVQDLLEQGRQHSQDLAFVSMLNDIAATPTAAMPFRGYTVLGVEGRVQEVQQVSTNKRPLWFICSGMGTQWRGMGLSLMRLDSFRESILRSDEAVKPLGVKVSDLLLSTDERTFDDIVHAFVSLTAIQIALIDLLTSVGLKPDGIIGHSLGEVACGYADGCLSQREAVLAAYWRGQCIKDAHLPPGSMAAVGLSWEECKQRCPAGVVPACHNSEDTVTISGPQAAVNEFVEQLKQEGVFAKEVRTGGLAFHSYFMEGIAPTLLQALKKVIREPRPRSARWLSTSIPEAQWQSSLARTSSAEYNVNNLVSPVLFQEALWHIPEHAVVLEIAPHALLQAVLKRGVKSSCTIIPLMKRDHKDNLEFFLTNLGKVHLTGINVNPNALFPPVEFPAPRGTPLISPHIKWDHSQTWDVPVAEDFPNGSSSSSATVYSIDASPESPDHYLVDHCIDGRVIFPGTGYLCLVWKTLARSLGLSLEETPVVFENVSFHQATILPKTGTVALEVRLLEASHAFEVSDTGNLIVSGKVYLWEDPNSKLFDHPEVPTPPESASVSRLTQGEVYKELRLRGYDYGPQFQGICEATLEGEQGKLLWKDNWVTFMDTMLQVSILGSSQQSLQLPTRVTAIYIDPATHRQKVYRLKEDTQVADVTTSRCLGITVSGGIHISRLQTTATSRRQQEQLVPTLEKFVFTPHMEAECLSESTALQKELQLCKGLARALQTKATQQGLKAAMLGQEDPPQHGLPRLLAAACQLQLNGNLQLELGEALAQERLLLPEDPLISGLLNSQALKACVDTALENLSTLKMKVAEVLAGEGHLYSRIPALLNTQPMLQLEYTATDRHPQALKDVQTKLQQHDVAQGQWNPSDPAPSSLGALDLLVCNCALATLGDPALALDNMVAALKEGGFLLVHTVLKGHALGETLACLPSEVQPAPSLLSQEEWESLFSRKALHLVGLKRSFYGTALFLCRRAIPQEKPIFLSVEDTSFQWVDSLKSTLATSSSQPVWLTAMDCPTSGVVGLVNCLRKEPGGHRIRCILLSNLSNTSHAPKLDPGSPELQQVLKHDLVMNVYRDGAWGAFRHFQLEQDKPKEQTAHAFVNVLTRGDLASIRWVSSPLKHTQPSSSGAQLCTVYYASLNFRDIMLATGKLSPDAIPGKWASRDCMLGMEFSGRDRCGRRVMGLVPAEGLATSVLLSSDFLWDVPSSWTLEEAASVPVVYTTAYYSLVVRGRIQRGETVLIHSGSGGVGQAAISIALSLGCRVFTTVGSAEKRAYLQARFPQLDDTSFANSRDTSFEQHVLLHTGGKGVDLVLNSLAEEKLQASVRCLAQHGRFLEIGKFDLSNNHPLGMAIFLKNVTFHGILLDALFEEANDSWREVAALLKAGIRDGVVKPLKCTVFPKAQVEDAFRYMAQGKHIGKVLVQVREEEPEAVLPGAQPTLISAISKTFCPAHKSYIITGGLGGFGLELARWLVLRGAQRLVLTSRSGIRTGYQAKHIREWRRQGIQVLVSTSNVSSLEGARALIAEATKLGPVGGVFNLAMVLRDAMLENQTPELFQDVNKPKYNGTLNLDRATREACPELDYFVAFSSVSCGRGNAGQTNYGFANSTMERICEQRRHDGLPGLAVQWGAIGDVGIVLEAMGTNDTVIGGTLPQRISSCMEVLDLFLNQPHAVLSSFVLAEKKAVAHGDGDTQRDLVKAVAHILGIRDLAGINLDSTLADLGLDSLMGVEVRQILEREHDLVLPMREVRQLTLRKLQEMSSKTDSATDTTAPKSRSDTSLKQNQAAAADTLLILGDSLSAGYRMSASAAWPALLNDKWQSKTSVVNASISGDTSQQGLARLPALLKQHQPRWVLVELGGNDGLRGFQPQQTEQTLRQILQDVKAANAEPLLMQIRLPANYGRRYNEAFSAIYPKLAKEFDVPLLPFFMEEVYLKPQWMQDDGIHPNRDAQPFIADWMAKQLQPLVNHDS

SEQ ID NO: 23 - protein, 2394 aa, synthetic construct
MEEVVIAGMSGKLPESENLQEFWANLIGGVDMVTDDDRRWKAGLYGLPKRSGKLKDLSKFDASFFGVHPKQAHTMDPQLRLLLEVSYEAIVDGGINPASLRGTNTGVWVGVSWSEASEALSRDPETLLGYSMVGCQRAMMANRLSFFFDFKGPSIALDTACSSSLLALQNAYQAIRSGECPAALVGGINLLLKPNTSVQFMKLGMLSPDGTCRSFDDSGSGYCRSEAVVAVLLTKKSLARRVYATILNAGTNTDGSKEQGVTFPSGEVQEQLICSLYQPAGLAPESLEYIEAHGTGTKVGDPQELNGITRSLCAFRQAPLLIGSTKSNMGHPEPASGLAALTKVLLSLEHGVWAPNLHFHNPNPEIPALLDGRLQVVDRPLPVRGGNVGINSFGFGGSNVHVILQPNTRQAPAPTAHAALPHLLHASGRTLEAVQDLLEQGRQHSQDLAFVSMLNDIAATPTAAMPFRGYTVLGVEGRVQEVQQVSTNKRPLWFICSGMGTQWRGMGLSLMRLDSFRESILRSDEAVKPLGVKVSDLLLSTDERTFDDIVHAFVSLTAIQIALIDLLTSVGLKPDGIIGHSLGEVACGYADGCLSQREAVLAAYWRGQCIKDAHLPPGSMAAVGLSWEECKQRCPAGVVPACHNSEDTVTISGPQAAVNEFVEQLKQEGVFAKEVRTGGLAFHSYFMEGIAPTLLQALKKVIREPRPRSARWLSTSIPEAQWQSSLARTSSAEYNVNNLVSPVLFQEALWHIPEHAVVLEIAPHALLQAVLKRGVKSSCTIIPLMKRDHKDNLEFFLTNLGKVHLTGINVNPNALFPPVEFPAPRGTPLISPHIKWDHSQTWDVPVAEDFPNGSSSSSATVYSIDASPESPDHYLVDHCIDGRVIFPGTGYLCLVWKTLARSLGLSLEETPVVFENVSFHQATILPKTGTVALEVRLLEASHAFEVSDTGNLIVSGKVYLWEDPNSKLFDHPEVPTPPESASVSRLTQGEVYKELRLRGYDYGPQFQGICEATLEGEQGKLLWKDNWVTFMDTMLQVSILGSSQQSLQLPTRVTAIYIDPATHRQKVYRLKEDTQVADVTTSRCLGITVSGGIHISRLQTTATSRRQQEQLVPTLEKFVFTPHMEAECLSESTALQKELQLCKGLARALQTKATQQGLKAAMLGQEDPPQHGLPRLLAAACQLQLNGNLQLELGEALAQERLLLPEDPLISGLLNSQALKACVDTALENLSTLKMKVAEVLAGEGHLYSRIPALLNTQPMLQLEYTATDRHPQALKDVQTKLQQHDVAQGQWNPSDPAPSSLGALDLLVCNCALATLGDPALALDNMVAALKEGGFLLVHTVLKGHALGETLACLPSEVQPAPSLLSQEEWESLFSRKALHLVGLKRSFYGTALFLCRRAIPQEKPIFLSVEDTSFQWVDSLKSTLATSSSQPVWLTAMDCPTSGVVGLVNCLRKEPGGHRIRCILLSNLSNTSHAPKLDPGSPELQQVLKHDLVMNVYRDGAWGAFRHFQLEQDKPKEQTAHAFVNVLTRGDLASIRWVSSPLKHTQPSSSGAQLCTVYYASLNFRDIMLATGKLSPDAIPGKWASRDCMLGMEFSGRDRCGRRVMGLVPAEGLATSVLLSSDFLWDVPSSWTLEEAASVPVVYTTAYYSLVVRGRIQRGETVLIHSGSGGVGQAAISIALSLGCRVFTTVGSAEKRAYLQARFPQLDDTSFANSRDTSFEQHVLLHTGGKGVDLVLNSLAEEKLQASVRCLAQHGRFLEIGKFDLSNNHPLGMAIFLKNVTFHGILLDALFEEANDSWREVAALLKAGIRDGVVKPLKCTVFPKAQVEDAFRYMAQGKHIGKVLVQVREEEPEAVLPGAQPTLISAISKTFCPAHKSYIITGGLGGFGLELARWLVLRGAQRLVLTSRSGIRTGYQAKHIREWRRQGIQVLVSTSNVSSLEGARALIAEATKLGPVGGVFNLAMVLRDAMLENQTPELFQDVNKPKYNGTLNLDRATREACPELDYFVAFSSVSCGRGNAGQTNYGFANSTMERICEQRRHDGLPGLAVQWGAIGDVGIVLEAMGTNDTVIGGTLPQRISSCMEVLDLFLNQPHAVLSSFVLAEKKAVAHGDGDTQRDLVKAVAHILGIRDLAGINLDSTLADLGLDSLMGVEVRQILEREHDLVLPMREVRQLTLRKLQEMSSKTDSATDTTAPKSRSDTSLKQNQAAAADTLLILGDSLSAGYRMSASAAWPALLNDKWQSKTSVVNASISGDTSQQGLARLPALLKQHQPRWVLVELGGNDGLRGFQPQQTEQTLRQILQDVKAANAEPLLMQIRPPANYGRRYNEAFSAIYPKLAKEFDVPLLPFFMEEVYLKPQWMQDDGIHPNRDAQPFIADWMAKQLQPLVNHDS

SEQ ID NO: 24 - protein, 2394 aa, synthetic construct
MEEVVIAGMSGKLPESENLQEFWANLIGGVDMVTDDDRRWKAGLYGLPKRSGKLKDLSKFDASFFGVHPKQAHTMDPQLRLLLEVSYEAIVDGGINPASLRGTNTGVWVGVSWSEASEALSRDPETLLGYSMVGCQRAMMANRLSFFFDFKGPSIALDTACSSSLLALQNAYQAIRSGECPAALVGGINLLLKPNTSVQFMKLGMLSPDGTCRSFDDSGSGYCRSEAVVAVLLTKKSLARRVYATILNAGTNTDGSKEQGVTFPSGEVQEQLICSLYQPAGLAPESLEYIEAHGTGTKVGDPQELNGITRSLCAFRQAPLLIGSTKSNMGHPEPASGLAALTKVLLSLEHGVWAPNLHFHNPNPEIPALLDGRLQVVDRPLPVRGGNVGINSFGFGGSNVHVILQPNTRQAPAPTAHAALPHLLHASGRTLEAVQDLLEQGRQHSQDLAFVSMLNDIAATPTAAMPFRGYTVLGVEGRVQEVQQVSTNKRPLWFICSGMGTQWRGMGLSLMRLDSFRESILRSDEAVKPLGVKVSDLLLSTDERTFDDIVHAFVSLTAIQIALIDLLTSVGLKPDGIIGHSLGEVACGYADGCLSQREAVLAAYWRGQCIKDAHLPPGSMAAVGLSWEECKQRCPAGVVPACHNSEDTVTISGPQAAVNEFVEQLKQEGVFAKEVRTGGLAFHSYFMEGIAPTLLQALKKVIREPRPRSARWLSTSIPEAQWQSSLARTSSAEYNVNNLVSPVLFQEALWHIPEHAVVLEIAPHALLQAVLKRGVKSSCTIIPLMKRDHKDNLEFFLTNLGKVHLTGINVNPNALFPPVEFPAPRGTPLISPHIKWDHSQTWDVPVAEDFPNGSSSSSATVYSIDASPESPDHYLVDHCIDGRVIFPGTGYLCLVWKTLARSLGLSLEETPVVFENVSFHQATILPKTGTVALEVRLLEASHAFEVSDTGNLIVSGKVYLWEDPNSKLFDHPEVPTPPESASVSRLTQGEVYKELRLRGYDYGPQFQGICEATLEGEQGKLLWKDNWVTFMDTMLQVSILGSSQQSLQLPTRVTAIYIDPATHRQKVYRLKEDTQVADVTTSRCLGITVSGGIHISRLQTTATSRRQQEQLVPTLEKFVFTPHMEAECLSESTALQKELQLCKGLARALQTKATQQGLKAAMLGQEDPPQHGLPRLLAAACQLQLNGNLQLELGEALAQERLLLPEDPLISGLLNSQALKACVDTALENLSTLKMKVAEVLAGEGHLYSRIPALLNTQPMLQLEYTATDRHPQALKDVQTKLQQHDVAQGQWNPSDPAPSSLGALDLLVCNCALATLGDPALALDNMVAALKEGGFLLVHTVLKGHALGETLACLPSEVQPAPSLLSQEEWESLFSRKALHLVGLKRSFYGTALFLCRRAIPQEKPIFLSVEDTSFQWVDSLKSTLATSSSQPVWLTAMDCPTSGVVGLVNCLRKEPGGHRIRCILLSNLSNTSHAPKLDPGSPELQQVLKHDLVMNVYRDGAWGAFRHFQLEQDKPKEQTAHAFVNVLTRGDLASIRWVSSPLKHTQPSSSGAQLCTVYYASLNFRDIMLATGKLSPDAIPGKWASRDCMLGMEFSGRDRCGRRVMGLVPAEGLATSVLLSSDFLWDVPSSWTLEEAASVPVVYTTAYYSLVVRGRIQRGETVLIHSGSGGVGQAAISIALSLGCRVFTTVGSAEKRAYLQARFPQLDDTSFANSRDTSFEQHVLLHTGGKGVDLVLNSLAEEKLQASVRCLAQHGRFLEIGKFDLSNNHPLGMAIFLKNVTFHGILLDALFEEANDSWREVAALLKAGIRDGVVKPLKCTVFPKAQVEDAFRYMAQGKHIGKVLVQVREEEPEAVLPGAQPTLISAISKTFCPAHKSYIITGGLGGFGLELARWLVLRGAQRLVLTSRSGIRTGYQAKHIREWRRQGIQVLVSTSNVSSLEGARALIAEATKLGPVGGVFNLAMVLRDAMLENQTPELFQDVNKPKYNGTLNLDRATREACPELDYFVAFSSVSCGRGNAGQTNYGFANSTMERICEQRRHDGLPGLAVQWGAIGDVGIVLEAMGTNDTVIGGTLPQRISSCMEVLDLFLNQPHAVLSSFVLAEKKAVAHGDGDTQRDLVKAVAHILGIRDLAGINLDSTLADLGLDSLMGVEVRQILEREHDLVLPMREVRQLTLRKLQEMSSKTDSATDTTAPKSRSDTSLKQNQAAAADTLLILGDSLSAGYRMSASAAWPALLNDKWQSKTSVVNASISGDTSQQGLARLPALLKQHQPRWVLVELGGNDGLRGFQPQQTEQTLRQILQDVKAANAEPLLMQIRLPANYGRRYNEAFSAIYPKLAKEFDVPLLPFFLDEVGKKPQWMQDDGIHPNRDAQPFIADWMAKQLQPLVNHDS

SEQ ID NO: 25 - protein, 2632 aa, synthetic construct
MEEVVIAGMSGKLPESENLQEFWANLIGGVDMVTDDDRRWKAGLYGLPKRSGKLKDLSKFDASFFGVHPKQAHTMDPQLRLLLEVSYEAIVDGGINPASLRGTNTGVWVGVSGSEASEALSRDPETLLGYSMVGCQRAMMANRLSFFFDFKGPSIALDTACSSSLLALQNAYQAIRSGECPAALVGGINLLLKPNTSVQFMKLGMLSPDGTCRSFDDSGSGYCRSEAVVAVLLTKKSLARRVYATILNAGTNTDGSKEQGVTFPSGEVQEQLICSLYQPAGLAPESLEYIEAHGTGTKVGDPQELNGITRSLCAFRQAPLLIGSTKSNMGHPEPASGLAALTKVLLSLEHGVWAPNLHFHNPNPEIPALLDGRLQVVDRPLPVRGGNVGINSFGFGGSNVHVILQPNTRQAPAPTAHAALPHLLHASGRTLEAVQDLLEQGRQHSQDLAFVSMLNDIAATPTAAMPFRGYTVLGVEGRVQEVQQVSTNKRPLWFICSGMGTQWRGMGLSLMRLDSFRESILRSDEAVKPLGVKVSDLLLSTDERTFDDIVHAFVSLTAIQIALIDLLTSVGLKPDGIIGHSLGEVACGYADGCLSQREAVLAAYWRGQCIKDAHLPPGSMAAVGLSWEECKQRCPAGVVPACHNSEDTVTISGPQAAVNEFVEQLKQEGVFAKEVRTGGLAFHSYFMEGIAPTLLQALKKVIREPRPRSARWLSTSIPEAQWQSSLARTSSAEYNVNNLVSPVLFQEALWHIPEHAVVLEIAPHALLQAVLKRGVKSSCTIIPLMKRDHKDNLEFFLTNLGKVHLTGINVNPNALFPPVEFPAPRGTPLISPHIKWDHSQTWDVPVAEDFPNGSSSSSATVYSIDASPESPDHYLVDHCIDGRVIFPGTGYLCLVWKTLARSLGLSLEETPVVFENVSFHQATILPKTGTVALEVRLLEASHAFEVSDTGNLIVSGKVYLWEDPNSKLFDHPEVPTPPESASVSRLTQGEVYKELRLRGYDYGPQFQGICEATLEGEQGKLLWKDNWVTFMDTMLQVSILGSSQQSLQLPTRVTAIYIDPATHRQKVYRLKEDTQVADVTTSRCLGITVSGGIHISRLQTTATSRRQQEQLVPTLEKFVFTPHMEAECLSESTALQKELQLCKGLARALQTKATQQGLKAAMLGQEDPPQHGLPRLLAAACQLQLNGNLQLELGEALAQERLLLPEDPLISGLLNSQALKACVDTALENLSTLKMKVAEVLAGEGHLYSRIPALLNTQPMLQLEYTATDRHPQALKDVQTKLQQHDVAQGQWNPSDPAPSSLGALDLLVCNCALATLGDPALALDNMVAALKEGGFLLVHTVLKGHALGETLACLPSEVQPAPSLLSQEEWESLFSRKALHLVGLKRSFYGTALFLCRRAIPQEKPIFLSVEDTSFQWVDSLKSTLATSSSQPVWLTAMDCPTSGVVGLVNCLRKEPGGHRIRCILLSNLSNTSHAPKLDPGSPELQQVLKHDLVMNVYRDGAWGAFRHFQLEQDKPKEQTAHAFVNVLTRGDLASIRWVSSPLKHTQPSSSGAQLCTVYYASLNFRDIMLATGKLSPDAIPGKWASRDCMLGMEFSGRDRCGRRVMGLVPAEGLATSVLLSSDFLWDVPSSWTLEEAASVPVVYTTAYYSLVVRGRIQRGETVLIHSGSGGVGQAAISIALSLGCRVFTTVGSAEKRAYLQARFPQLDDTSFANSRDTSFEQHVLLHTGGKGVDLVLNSLAEEKLQASVRCLAQHGRFLEIGKFDLSNNHPLGMAIFLKNVTFHGILLDALFEEANDSWREVAALLKAGIRDGVVKPLKCTVFPKAQVEDAFRYMAQGKHIGKVLVQVREEEPEAVLPGAQPTLISAISKTFCPAHKSYIITGGLGGFGLELARWLVLRGAQRLVLTSRSGIRTGYQAKHIREWRRQGIQVLVSTSNVSSLEGARALIAEATKLGPVGGVFNLAMVLRDAMLENQTPELFQDVNKPKYNGTLNLDRATREACPELDYFVAFSSVSCGRGNAGQTNYGFANSTMERICEQRRHDGLPGLAVQWGAIGDVGIVLEAMGTNDTVIGGTLPQRISSCMEVLDLFLNQPHAVLSSFVLAEKKAVAHGDGDTQRDLVKAVAHILGIRDLAGINLDSTLADLGLDSLMGVEVRQILEREHDLVLPMREVRQLTLRKLQEMSSKAAAAQRTAGDRRPSFTTVHGADATEIRASELTLDKFIDAETLRAAPGLPKVTTEPRTVLLSGANGWLGRFLTLQWLERLAPVGGTLITIVRGRDDAAARARLTQAYDTDPELSRRFAELADRHLRVVAGDIGDPNLGLTPEIWHRLAAEVDLVVHPAALVNHVLPYRQLFGPNVVGTAEVIKLALTERIKPVTYLSTVSVAMGIPDFEEDGDIRTVSPVRPLDGGYANGYGNSKWAGEVLLREAHDLCGLPVATFRSDMILAHPRYRGQVNVPDMFTRLLLSLLITGVAPRSFYIGDGERPRAHYPGLTVDFVAEAVTTLGAQQREGYVSYDVMNPHDDGISLDVFVDWLIRAGHPIDRVDDYDDWVRRFETALTALPEKRRAQTVLPLLHAFRAPQAPLRGAPEPTEVFHAAVRTAKVGPGDIPHLDEALIDKYIRDLREFGLI

SEQ ID NO: 26 - protein, 2643 aa, synthetic construct
MEEVVIAGMSGKLPESENLQEFWANLIGGVDMVTDDDRRWKAGLYGLPKRSGKLKDLSKFDASFFGVHPKQAHTMDPQLRLLLEVSYEAIVDGGINPASLRGTNTGVWVGVSGSEASEALSRDPETLLGYSMVGCQRAMMANRLSFFFDFKGPSIALDTACSSSLLALQNAYQAIRSGECPAALVGGINLLLKPNTSVQFMKLGMLSPDGTCRSFDDSGSGYCRSEAVVAVLLTKKSLARRVYATILNAGTNTDGSKEQGVTFPSGEVQEQLICSLYQPAGLAPESLEYIEAHGTGTKVGDPQELNGITRSLCAFRQAPLLIGSTKSNMGHPEPASGLAALTKVLLSLEHGVWAPNLHFHNPNPEIPALLDGRLQVVDRPLPVRGGNVGINSFGFGGSNVHVILQPNTRQAPAPTAHAALPHLLHASGRTLEAVQDLLEQGRQHSQDLAFVSMLNDIAATPTAAMPFRGYTVLGVEGRVQEVQQVSTNKRPLWFICSGMGTQWRGMGLSLMRLDSFRESILRSDEAVKPLGVKVSDLLLSTDERTFDDIVHAFVSLTAIQIALIDLLTSVGLKPDGIIGHSLGEVACGYADGCLSQREAVLAAYWRGQCIKDAHLPPGSMAAVGLSWEECKQRCPAGVVPACHNSEDTVTISGPQAAVNEFVEQLKQEGVFAKEVRTGGLAFHSYFMEGIAPTLLQALKKVIREPRPRSARWLSTSIPEAQWQSSLARTSSAEYNVNNLVSPVLFQEALWHIPEHAVVLEIAPHALLQAVLKRGVKSSCTIIPLMKRDHKDNLEFFLTNLGKVHLTGINVNPNALFPPVEFPAPRGTPLISPHIKWDHSQTWDVPVAEDFPNGSSSSSATVYSIDASPESPDHYLVDHCIDGRVIFPGTGYLCLVWKTLARSLGLSLEETPVVFENVSFHQATILPKTGTVALEVRLLEASHAFEVSDTGNLIVSGKVYLWEDPNSKLFDHPEVPTPPESASVSRLTQGEVYKELRLRGYDYGPQFQGICEATLEGEQGKLLWKDNWVTFMDTMLQVSILGSSQQSLQLPTRVTAIYIDPATHRQKVYRLKEDTQVADVTTSRCLGITVSGGIHISRLQTTATSRRQQEQLVPTLEKFVFTPHMEAECLSESTALQKELQLCKGLARALQTKATQQGLKAAMLGQEDPPQHGLPRLLAAACQLQLNGNLQLELGEALAQERLLLPEDPLISGLLNSQALKACVDTALENLSTLKMKVAEVLAGEGHLYSRIPALLNTQPMLQLEYTATDRHPQALKDVQTKLQQHDVAQGQWNPSDPAPSSLGALDLLVCNCALATLGDPALALDNMVAALKEGGFLLVHTVLKGHALGETLACLPSEVQPAPSLLSQEEWESLFSRKALHLVGLKRSFYGTALFLCRRAIPQEKPIFLSVEDTSFQWVDSLKSTLATSSSQPVWLTAMDCPTSGVVGLVNCLRKEPGGHRIRCILLSNLSNTSHAPKLDPGSPELQQVLKHDLVMNVYRDGAWGAFRHFQLEQDKPKEQTAHAFVNVLTRGDLASIRWVSSPLKHTQPSSSGAQLCTVYYASLNFRDIMLATGKLSPDAIPGKWASRDCMLGMEFSGRDRCGRRVMGLVPAEGLATSVLLSSDFLWDVPSSWTLEEAASVPVVYTTAYYSLVVRGRIQRGETVLIHSGSGGVGQAAISIALSLGCRVFTTVGSAEKRAYLQARFPQLDDTSFANSRDTSFEQHVLLHTGGKGVDLVLNSLAEEKLQASVRCLAQHGRFLEIGKFDLSNNHPLGMAIFLKNVTFHGILLDALFEEANDSWREVAALLKAGIRDGVVKPLKCTVFPKAQVEDAFRYMAQGKHIGKVLVQVREEEPEAVLPGAQPTLISAISKTFCPAHKSYIITGGLGGFGLELARWLVLRGAQRLVLTSRSGIRTGYQAKHIREWRRQGIQVLVSTSNVSSLEGARALIAEATKLGPVGGVFNLAMVLRDAMLENQTPELFQDVNKPKYNGTLNLDRATREACPELDYFVAFSSVSCGRGNAGQTNYGFANSTMERICEQRRHDGLPGLAVQWGAIGDVGIVLEAMGTNDTVIGGTLPQRISSCMEVLDLFLNQPHAVLSSFVLAEKKAVAHGDGDTQRDLVKAVAHILGIRDLAGINLDSTLADLGLDSLMGVEVRQILEREHDLVLPMREVRQLTLRKLQEMSSKTDSAAATARRPGDGRPTFAGVHGDDAAEVHARDLTLDRFLDDATLAAATALPGPAPEIRTVLLTGATGFLGRYLALEWLERMAMVGGTLICLVRGRDDAAARARLDQIFDSGDPELLRHYRELADRHLEVIAGDKSDAVLGLDRRTWQRLADTVDLIVDPAALVNHVLPYRELFGPNVVGTAELIRLALTGRLKPYLYTSTIAVGAGIAPGQFTEDADIRQISATRTLDDSYANGYATSKWAGEVLLREAHDLCGLPVAVFRCDMILADTSYAGQLNVPDMFTRLILSLVATGIAPLSFYELDAAGHRQRAHYDGLPVEFVAEAVSALGLDVAEDGGFATYHVMNPYDDGIGLDEFVDWLTGAGYPIERVNDYGTWFQRFETAIRGLPERQRQASLLPLLHNYQRPQPPIRGSAAPTDRFRSAVQDAKIGPDKDIPHITPEVIVKYVTDLRLLGLL

SEQ ID NO: 27 - protein, 2639 aa, synthetic construct
MEEVVIAGMSGKLPESENLQEFWANLIGGVDMVTDDDRRWKAGLYGLPKRSGKLKDLSKFDASFFGVHPKQAHTMDPQLRLLLEVSYEAIVDGGINPASLRGTNTGVWVGVSGSEASEALSRDPETLLGYSMVGCQRAMMANRLSFFFDFKGPSIALDTACSSSLLALQNAYQAIRSGECPAALVGGINLLLKPNTSVQFMKLGMLSPDGTCRSFDDSGSGYCRSEAVVAVLLTKKSLARRVYATILNAGTNTDGSKEQGVTFPSGEVQEQLICSLYQPAGLAPESLEYIEAHGTGTKVGDPQELNGITRSLCAFRQAPLLIGSTKSNMGHPEPASGLAALTKVLLSLEHGVWAPNLHFHNPNPEIPALLDGRLQVVDRPLPVRGGNVGINSFGFGGSNVHVILQPNTRQAPAPTAHAALPHLLHASGRTLEAVQDLLEQGRQHSQDLAFVSMLNDIAATPTAAMPFRGYTVLGVEGRVQEVQQVSTNKRPLWFICSGMGTQWRGMGLSLMRLDSFRESILRSDEAVKPLGVKVSDLLLSTDERTFDDIVHAFVSLTAIQIALIDLLTSVGLKPDGIIGHSLGEVACGYADGCLSQREAVLAAYWRGQCIKDAHLPPGSMAAVGLSWEECKQRCPAGVVPACHNSEDTVTISGPQAAVNEFVEQLKQEGVFAKEVRTGGLAFHSYFMEGIAPTLLQALKKVIREPRPRSARWLSTSIPEAQWQSSLARTSSAEYNVNNLVSPVLFQEALWHIPEHAVVLEIAPHALLQAVLKRGVKSSCTIIPLMKRDHKDNLEFFLTNLGKVHLTGINVNPNALFPPVEFPAPRGTPLISPHIKWDHSQTWDVPVAEDFPNGSSSSSATVYSIDASPESPDHYLVDHCIDGRVIFPGTGYLCLVWKTLARSLGLSLEETPVVFENVSFHQATILPKTGTVALEVRLLEASHAFEVSDTGNLIVSGKVYLWEDPNSKLFDHPEVPTPPESASVSRLTQGEVYKELRLRGYDYGPQFQGICEATLEGEQGKLLWKDNWVTFMDTMLQVSILGSSQQSLQLPTRVTAIYIDPATHRQKVYRLKEDTQVADVTTSRCLGITVSGGIHISRLQTTATSRRQQEQLVPTLEKFVFTPHMEAECLSESTALQKELQLCKGLARALQTKATQQGLKAAMLGQEDPPQHGLPRLLAAACQLQLNGNLQLELGEALAQERLLLPEDPLISGLLNSQALKACVDTALENLSTLKMKVAEVLAGEGHLYSRIPALLNTQPMLQLEYTATDRHPQALKDVQTKLQQHDVAQGQWNPSDPAPSSLGALDLLVCNCALATLGDPALALDNMVAALKEGGFLLVHTVLKGHALGETLACLPSEVQPAPSLLSQEEWESLFSRKALHLVGLKRSFYGTALFLCRRAIPQEKPIFLSVEDTSFQWVDSLKSTLATSSSQPVWLTAMDCPTSGVVGLVNCLRKEPGGHRIRCILLSNLSNTSHAPKLDPGSPELQQVLKHDLVMNVYRDGAWGAFRHFQLEQDKPKEQTAHAFVNVLTRGDLASIRWVSSPLKHTQPSSSGAQLCTVYYASLNFRDIMLATGKLSPDAIPGKWASRDCMLGMEFSGRDRCGRRVMGLVPAEGLATSVLLSSDFLWDVPSSWTLEEAASVPVVYTTAYYSLVVRGRIQRGETVLIHSGSGGVGQAAISIALSLGCRVFTTVGSAEKRAYLQARFPQLDDTSFANSRDTSFEQHVLLHTGGKGVDLVLNSLAEEKLQASVRCLAQHGRFLEIGKFDLSNNHPLGMAIFLKNVTFHGILLDALFEEANDSWREVAALLKAGIRDGVVKPLKCTVFPKAQVEDAFRYMAQGKHIGKVLVQVREEEPEAVLPGAQPTLISAISKTFCPAHKSYIITGGLGGFGLELARWLVLRGAQRLVLTSRSGIRTGYQAKHIREWRRQGIQVLVSTSNVSSLEGARALIAEATKLGPVGGVFNLAMVLRDAMLENQTPELFQDVNKPKYNGTLNLDRATREACPELDYFVAFSSVSCGRGNAGQTNYGFANSTMERICEQRRHDGLPGLAVQWGAIGDVGIVLEAMGTNDTVIGGTLPQRISSCMEVLDLFLNQPHAVLSSFVLAEKKAVAHGDGDTQRDLVKAVAHILGIRDLAGINLDSTLADLGLDSLMGVEVRQILEREHDLVLPMREVRQLTLRKLQEMSSKTDSAAASERDSGSRPTAATVHGDDGLLRADDLALEAFLDPATLDAAAHLPSALEPPRTVLLTGANGYLGRFLALEWLQRLDVSGGTLICLIRGSDADSARRRLDAVFATGDPELEAHYRELAERRLRVLPGDIGEPNLGLREQDWRDLAETVDLIVHPAALVNHVLPYAQLFGPNVVGTAEVIRLALTSRLKPVTYLSTVAVSAGIDPETFTEDGDIREISPVRRLDDGYANGYGNSKWAGEVLLRNAHDRFGLPVAVFRSDMILAHSRYAGQLNVPDMFTRLLLSVLATGLAPGSFHDAHGERHRAHYDGLPADFTAAAVTTLGSRVTSGYETYDVLNPHDDGISLDTFVDWLIEAGHPIDRIDDYAEWFARFDTALRALPEHQRQHSLLPLLHAYRRPTPPLHGVALPAKHFRAAVQQAKLGPDGDIPHVTRELIEKYASDLRLLGLIQG

SEQ ID NO: 28 - protein, 2632 aa, synthetic construct
MEEVVIAGMSGKLPESENLQEFWANLIGGVDMVTDDDRRWKAGLYGLPKRSGKLKDLSKFDASFFGVHPKQAHTMDPQLRLLLEVSYEAIVDGGINPASLRGTNTGVWVGVSWSEASEALSRDPETLLGYSMVGCQRAMMANRLSFFFDFKGPSIALDTACSSSLLALQNAYQAIRSGECPAALVGGINLLLKPNTSVQFMKLGMLSPDGTCRSFDDSGSGYCRSEAVVAVLLTKKSLARRVYATILNAGTNTDGSKEQGVTFPSGEVQEQLICSLYQPAGLAPESLEYIEAHGTGTKVGDPQELNGITRSLCAFRQAPLLIGSTKSNMGHPEPASGLAALTKVLLSLEHGVWAPNLHFHNPNPEIPALLDGRLQVVDRPLPVRGGNVGINSFGFGGSNVHVILQPNTRQAPAPTAHAALPHLLHASGRTLEAVQDLLEQGRQHSQDLAFVSMLNDIAATPTAAMPFRGYTVLGVEGRVQEVQQVSTNKRPLWFICSGMGTQWRGMGLSLMRLDSFRESILRSDEAVKPLGVKVSDLLLSTDERTFDDIVHAFVSLTAIQIALIDLLTSVGLKPDGIIGHSLGEVACGYADGCLSQREAVLAAYWRGQCIKDAHLPPGSMAAVGLSWEECKQRCPAGVVPACHNSEDTVTISGPQAAVNEFVEQLKQEGVFAKEVRTGGLAFHSYFMEGIAPTLLQALKKVIREPRPRSARWLSTSIPEAQWQSSLARTSSAEYNVNNLVSPVLFQEALWHIPEHAVVLEIAPHALLQAVLKRGVKSSCTIIPLMKRDHKDNLEFFLTNLGKVHLTGINVNPNALFPPVEFPAPRGTPLISPHIKWDHSQTWDVPVAEDFPNGSSSSSATVYSIDASPESPDHYLVDHCIDGRVIFPGTGYLCLVWKTLARSLGLSLEETPVVFENVSFHQATILPKTGTVALEVRLLEASHAFEVSDTGNLIVSGKVYLWEDPNSKLFDHPEVPTPPESASVSRLTQGEVYKELRLRGYDYGPQFQGICEATLEGEQGKLLWKDNWVTFMDTMLQVSILGSSQQSLQLPTRVTAIYIDPATHRQKVYRLKEDTQVADVTTSRCLGITVSGGIHISRLQTTATSRRQQEQLVPTLEKFVFTPHMEAECLSESTALQKELQLCKGLARALQTKATQQGLKAAMLGQEDPPQHGLPRLLAAACQLQLNGNLQLELGEALAQERLLLPEDPLISGLLNSQALKACVDTALENLSTLKMKVAEVLAGEGHLYSRIPALLNTQPMLQLEYTATDRHPQALKDVQTKLQQHDVAQGQWNPSDPAPSSLGALDLLVCNCALATLGDPALALDNMVAALKEGGFLLVHTVLKGHALGETLACLPSEVQPAPSLLSQEEWESLFSRKALHLVGLKRSFYGTALFLCRRAIPQEKPIFLSVEDTSFQWVDSLKSTLATSSSQPVWLTAMDCPTSGVVGLVNCLRKEPGGHRIRCILLSNLSNTSHAPKLDPGSPELQQVLKHDLVMNVYRDGAWGAFRHFQLEQDKPKEQTAHAFVNVLTRGDLASIRWVSSPLKHTQPSSSGAQLCTVYYASLNFRDIMLATGKLSPDAIPGKWASRDCMLGMEFSGRDRCGRRVMGLVPAEGLATSVLLSSDFLWDVPSSWTLEEAASVPVVYTTAYYSLVVRGRIQRGETVLIHSGSGGVGQAAISIALSLGCRVFTTVGSAEKRAYLQARFPQLDDTSFANSRDTSFEQHVLLHTGGKGVDLVLNSLAEEKLQASVRCLAQHGRFLEIGKFDLSNNHPLGMAIFLKNVTFHGILLDALFEEANDSWREVAALLKAGIRDGVVKPLKCTVFPKAQVEDAFRYMAQGKHIGKVLVQVREEEPEAVLPGAQPTLISAISKTFCPAHKSYIITGGLGGFGLELARWLVLRGAQRLVLTSRSGIRTGYQAKHIREWRRQGIQVLVSTSNVSSLEGARALIAEATKLGPVGGVFNLAMVLRDAMLENQTPELFQDVNKPKYNGTLNLDRATREACPELDYFVAFSSVSCGRGNAGQTNYGFANSTMERICEQRRHDGLPGLAVQWGAIGDVGIVLEAMGTNDTVIGGTLPQRISSCMEVLDLFLNQPHAVLSSFVLAEKKAVAHGDGDTQRDLVKAVAHILGIRDLAGINLDSTLADLGLDSLMGVEVRQILEREHDLVLPMREVRQLTLRKLQEMSSKAAAAQRTAGDRRPSFTTVHGADATEIRASELTLDKFIDAETLRAAPGLPKVTTEPRTVLLSGANGWLGRFLTLQWLERLAPVGGTLITIVRGRDDAAARARLTQAYDTDPELSRRFAELADRHLRVVAGDIGDPNLGLTPEIWHRLAAEVDLVVHPAALVNHVLPYRQLFGPNVVGTAEVIKLALTERIKPVTYLSTVSVAMGIPDFEEDGDIRTVSPVRPLDGGYANGYGNSKWAGEVLLREAHDLCGLPVATFRSDMILAHPRYRGQVNVPDMFTRLLLSLLITGVAPRSFYIGDGERPRAHYPGLTVDFVAEAVTTLGAQQREGYVSYDVMNPHDDGISLDVFVDWLIRAGHPIDRVDDYDDWVRRFETALTALPEKRRAQTVLPLLHAFRAPQAPLRGAPEPTEVFHAAVRTAKVGPGDIPHLDEALIDKYIRDLREFGLI

SEQ ID NO: 29 - protein, 2643 aa, synthetic construct
MEEVVIAGMSGKLPESENLQEFWANLIGGVDMVTDDDRRWKAGLYGLPKRSGKLKDLSKFDASFFGVHPKQAHTMDPQLRLLLEVSYEAIVDGGINPASLRGTNTGVWVGVSWSEASEALSRDPETLLGYSMVGCQRAMMANRLSFFFDFKGPSIALDTACSSSLLALQNAYQAIRSGECPAALVGGINLLLKPNTSVQFMKLGMLSPDGTCRSFDDSGSGYCRSEAVVAVLLTKKSLARRVYATILNAGTNTDGSKEQGVTFPSGEVQEQLICSLYQPAGLAPESLEYIEAHGTGTKVGDPQELNGITRSLCAFRQAPLLIGSTKSNMGHPEPASGLAALTKVLLSLEHGVWAPNLHFHNPNPEIPALLDGRLQVVDRPLPVRGGNVGINSFGFGGSNVHVILQPNTRQAPAPTAHAALPHLLHASGRTLEAVQDLLEQGRQHSQDLAFVSMLNDIAATPTAAMPFRGYTVLGVEGRVQEVQQVSTNKRPLWFICSGMGTQWRGMGLSLMRLDSFRESILRSDEAVKPLGVKVSDLLLSTDERTFDDIVHAFVSLTAIQIALIDLLTSVGLKPDGIIGHSLGEVACGYADGCLSQREAVLAAYWRGQCIKDAHLPPGSMAAVGLSWEECKQRCPAGVVPACHNSEDTVTISGPQAAVNEFVEQLKQEGVFAKEVRTGGLAFHSYFMEGIAPTLLQALKKVIREPRPRSARWLSTSIPEAQWQSSLARTSSAEYNVNNLVSPVLFQEALWHIPEHAVVLEIAPHALLQAVLKRGVKSSCTIIPLMKRDHKDNLEFFLTNLGKVHLTGINVNPNALFPPVEFPAPRGTPLISPHIKWDHSQTWDVPVAEDFPNGSSSSSATVYSIDASPESPDHYLVDHCIDGRVIFPGTGYLCLVWKTLARSLGLSLEETPVVFENVSFHQATILPKTGTVALEVRLLEASHAFEVSDTGNLIVSGKVYLWEDPNSKLFDHPEVPTPPESASVSRLTQGEVYKELRLRGYDYGPQFQGICEATLEGEQGKLLWKDNWVTFMDTMLQVSILGSSQQSLQLPTRVTAIYIDPATHRQKVYRLKEDTQVADVTTSRCLGITVSGGIHISRLQTTATSRRQQEQLVPTLEKFVFTPHMEAECLSESTALQKELQLCKGLARALQTKATQQGLKAAMLGQEDPPQHGLPRLLAAACQLQLNGNLQLELGEALAQERLLLPEDPLISGLLNSQALKACVDTALENLSTLKMKVAEVLAGEGHLYSRIPALLNTQPMLQLEYTATDRHPQALKDVQTKLQQHDVAQGQWNPSDPAPSSLGALDLLVCNCALATLGDPALALDNMVAALKEGGFLLVHTVLKGHALGETLACLPSEVQPAPSLLSQEEWESLFSRKALHLVGLKRSFYGTALFLCRRAIPQEKPIFLSVEDTSFQWVDSLKSTLATSSSQPVWLTAMDCPTSGVVGLVNCLRKEPGGHRIRCILLSNLSNTSHAPKLDPGSPELQQVLKHDLVMNVYRDGAWGAFRHFQLEQDKPKEQTAHAFVNVLTRGDLASIRWVSSPLKHTQPSSSGAQLCTVYYASLNFRDIMLATGKLSPDAIPGKWASRDCMLGMEFSGRDRCGRRVMGLVPAEGLATSVLLSSDFLWDVPSSWTLEEAASVPVVYTTAYYSLVVRGRIQRGETVLIHSGSGGVGQAAISIALSLGCRVFTTVGSAEKRAYLQARFPQLDDTSFANSRDTSFEQHVLLHTGGKGVDLVLNSLAEEKLQASVRCLAQHGRFLEIGKFDLSNNHPLGMAIFLKNVTFHGILLDALFEEANDSWREVAALLKAGIRDGVVKPLKCTVFPKAQVEDAFRYMAQGKHIGKVLVQVREEEPEAVLPGAQPTLISAISKTFCPAHKSYIITGGLGGFGLELARWLVLRGAQRLVLTSRSGIRTGYQAKHIREWRRQGIQVLVSTSNVSSLEGARALIAEATKLGPVGGVFNLAMVLRDAMLENQTPELFQDVNKPKYNGTLNLDRATREACPELDYFVAFSSVSCGRGNAGQTNYGFANSTMERICEQRRHDGLPGLAVQWGAIGDVGIVLEAMGTNDTVIGGTLPQRISSCMEVLDLFLNQPHAVLSSFVLAEKKAVAHGDGDTQRDLVKAVAHILGIRDLAGINLDSTLADLGLDSLMGVEVRQILEREHDLVLPMREVRQLTLRKLQEMSSKTDSAAATARRPGDGRPTFAGVHGDDAAEVHARDLTLDRFLDDATLAAATALPGPAPEIRTVLLTGATGFLGRYLALEWLERMAMVGGTLICLVRGRDDAAARARLDQIFDSGDPELLRHYRELADRHLEVIAGDKSDAVLGLDRRTWQRLADTVDLIVDPAALVNHVLPYRELFGPNVVGTAELIRLALTGRLKPYLYTSTIAVGAGIAPGQFTEDADIRQISATRTLDDSYANGYATSKWAGEVLLREAHDLCGLPVAVFRCDMILADTSYAGQLNVPDMFTRLILSLVATGIAPLSFYELDAAGHRQRAHYDGLPVEFVAEAVSALGLDVAEDGGFATYHVMNPYDDGIGLDEFVDWLTGAGYPIERVNDYGTWFQRFETAIRGLPERQRQASLLPLLHNYQRPQPPIRGSAAPTDRFRSAVQDAKIGPDKDIPHITPEVIVKYVTDLRLLGLL

SEQ ID NO: 30 - protein, 2639 aa, synthetic construct
MEEVVIAGMSGKLPESENLQEFWANLIGGVDMVTDDDRRWKAGLYGLPKRSGKLKDLSKFDASFFGVHPKQAHTMDPQLRLLLEVSYEAIVDGGINPASLRGTNTGVWVGVSWSEASEALSRDPETLLGYSMVGCQRAMMANRLSFFFDFKGPSIALDTACSSSLLALQNAYQAIRSGECPAALVGGINLLLKPNTSVQFMKLGMLSPDGTCRSFDDSGSGYCRSEAVVAVLLTKKSLARRVYATILNAGTNTDGSKEQGVTFPSGEVQEQLICSLYQPAGLAPESLEYIEAHGTGTKVGDPQELNGITRSLCAFRQAPLLIGSTKSNMGHPEPASGLAALTKVLLSLEHGVWAPNLHFHNPNPEIPALLDGRLQVVDRPLPVRGGNVGINSFGFGGSNVHVILQPNTRQAPAPTAHAALPHLLHASGRTLEAVQDLLEQGRQHSQDLAFVSMLNDIAATPTAAMPFRGYTVLGVEGRVQEVQQVSTNKRPLWFICSGMGTQWRGMGLSLMRLDSFRESILRSDEAVKPLGVKVSDLLLSTDERTFDDIVHAFVSLTAIQIALIDLLTSVGLKPDGIIGHSLGEVACGYADGCLSQREAVLAAYWRGQCIKDAHLPPGSMAAVGLSWEECKQRCPAGVVPACHNSEDTVTISGPQAAVNEFVEQLKQEGVFAKEVRTGGLAFHSYFMEGIAPTLLQALKKVIREPRPRSARWLSTSIPEAQWQSSLARTSSAEYNVNNLVSPVLFQEALWHIPEHAVVLEIAPHALLQAVLKRGVKSSCTIIPLMKRDHKDNLEFFLTNLGKVHLTGINVNPNALFPPVEFPAPRGTPLISPHIKWDHSQTWDVPVAEDFPNGSSSSSATVYSIDASPESPDHYLVDHCIDGRVIFPGTGYLCLVWKTLARSLGLSLEETPVVFENVSFHQATILPKTGTVALEVRLLEASHAFEVSDTGNLIVSGKVYLWEDPNSKLFDHPEVPTPPESASVSRLTQGEVYKELRLRGYDYGPQFQGICEATLEGEQGKLLWKDNWVTFMDTMLQVSILGSSQQSLQLPTRVTAIYIDPATHRQKVYRLKEDTQVADVTTSRCLGITVSGGIHISRLQTTATSRRQQEQLVPTLEKFVFTPHMEAECLSESTALQKELQLCKGLARALQTKATQQGLKAAMLGQEDPPQHGLPRLLAAACQLQLNGNLQLELGEALAQERLLLPEDPLISGLLNSQALKACVDTALENLSTLKMKVAEVLAGEGHLYSRIPALLNTQPMLQLEYTATDRHPQALKDVQTKLQQHDVAQGQWNPSDPAPSSLGALDLLVCNCALATLGDPALALDNMVAALKEGGFLLVHTVLKGHALGETLACLPSEVQPAPSLLSQEEWESLFSRKALHLVGLKRSFYGTALFLCRRAIPQEKPIFLSVEDTSFQWVDSLKSTLATSSSQPVWLTAMDCPTSGVVGLVNCLRKEPGGHRIRCILLSNLSNTSHAPKLDPGSPELQQVLKHDLVMNVYRDGAWGAFRHFQLEQDKPKEQTAHAFVNVLTRGDLASIRWVSSPLKHTQPSSSGAQLCTVYYASLNFRDIMLATGKLSPDAIPGKWASRDCMLGMEFSGRDRCGRRVMGLVPAEGLATSVLLSSDFLWDVPSSWTLEEAASVPVVYTTAYYSLVVRGRIQRGETVLIHSGSGGVGQAAISIALSLGCRVFTTVGSAEKRAYLQARFPQLDDTSFANSRDTSFEQHVLLHTGGKGVDLVLNSLAEEKLQASVRCLAQHGRFLEIGKFDLSNNHPLGMAIFLKNVTFHGILLDALFEEANDSWREVAALLKAGIRDGVVKPLKCTVFPKAQVEDAFRYMAQGKHIGKVLVQVREEEPEAVLPGAQPTLISAISKTFCPAHKSYIITGGLGGFGLELARWLVLRGAQRLVLTSRSGIRTGYQAKHIREWRRQGIQVLVSTSNVSSLEGARALIAEATKLGPVGGVFNLAMVLRDAMLENQTPELFQDVNKPKYNGTLNLDRATREACPELDYFVAFSSVSCGRGNAGQTNYGFANSTMERICEQRRHDGLPGLAVQWGAIGDVGIVLEAMGTNDTVIGGTLPQRISSCMEVLDLFLNQPHAVLSSFVLAEKKAVAHGDGDTQRDLVKAVAHILGIRDLAGINLDSTLADLGLDSLMGVEVRQILEREHDLVLPMREVRQLTLRKLQEMSSKTDSAAASERDSGSRPTAATVHGDDGLLRADDLALEAFLDPATLDAAAHLPSALEPPRTVLLTGANGYLGRFLALEWLQRLDVSGGTLICLIRGSDADSARRRLDAVFATGDPELEAHYRELAERRLRVLPGDIGEPNLGLREQDWRDLAETVDLIVHPAALVNHVLPYAQLFGPNVVGTAEVIRLALTSRLKPVTYLSTVAVSAGIDPETFTEDGDIREISPVRRLDDGYANGYGNSKWAGEVLLRNAHDRFGLPVAVFRSDMILAHSRYAGQLNVPDMFTRLLLSVLATGLAPGSFHDAHGERHRAHYDGLPADFTAAAVTTLGSRVTSGYETYDVLNPHDDGISLDTFVDWLIEAGHPIDRIDDYAEWFARFDTALRALPEHQRQHSLLPLLHAYRRPTPPLHGVALPAKHFRAAVQQAKLGPDGDIPHVTRELIEKYASDLRLLGLIQG

SEQ ID NO: 31 - protein, 2394 aa, synthetic construct
MEEVVIAGMSGKLPESENLQEFWANLIGGVDMVTDDDRRWKAGLYGLPKRSGKLKDLSKFDASFFGVHPKQAHTMDPQLRLLLEVSYEAIVDGGINPASLRGTNTGVWVGVSTSEASEALSRDPETLLGYSMVGCQRAMMANRLSFFFDFKGPSIALDTACSSSLLALQNAYQAIRSGECPAALVGGINLLLKPNTSVQFMKLGMLSPDGTCRSFDDSGSGYCRSEAVVAVLLTKKSLARRVYATILNAGTNTDGSKEQGVTFPSGEVQEQLICSLYQPAGLAPESLEYIEAHGTGTKVGDPQELNGITRSLCAFRQAPLLIGSTKSNMGHPEPASGLAALTKVLLSLEHGVWAPNLHFHNPNPEIPALLDGRLQVVDRPLPVRGGNVGINSFGFGGSNVHVILQPNTRQAPAPTAHAALPHLLHASGRTLEAVQDLLEQGRQHSQDLAFVSMLNDIAATPTAAMPFRGYTVLGVEGRVQEVQQVSTNKRPLWFICSGMGTQWRGMGLSLMRLDSFRESILRSDEAVKPLGVKVSDLLLSTDERTFDDIVHAFVSLTAIQIALIDLLTSVGLKPDGIIGHSLGEVACGYADGCLSQREAVLAAYWRGQCIKDAHLPPGSMAAVGLSWEECKQRCPAGVVPACHNSEDTVTISGPQAAVNEFVEQLKQEGVFAKEVRTGGLAFHSYFMEGIAPTLLQALKKVIREPRPRSARWLSTSIPEAQWQSSLARTSSAEYNVNNLVSPVLFQEALWHIPEHAVVLEIAPHALLQAVLKRGVKSSCTIIPLMKRDHKDNLEFFLTNLGKVHLTGINVNPNALFPPVEFPAPRGTPLISPHIKWDHSQTWDVPVAEDFPNGSSSSSATVYSIDASPESPDHYLVDHCIDGRVIFPGTGYLCLVWKTLARSLGLSLEETPVVFENVSFHQATILPKTGTVALEVRLLEASHAFEVSDTGNLIVSGKVYLWEDPNSKLFDHPEVPTPPESASVSRLTQGEVYKELRLRGYDYGPQFQGICEATLEGEQGKLLWKDNWVTFMDTMLQVSILGSSQQSLQLPTRVTAIYIDPATHRQKVYRLKEDTQVADVTTSRCLGITVSGGIHISRLQTTATSRRQQEQLVPTLEKFVFTPHMEAECLSESTALQKELQLCKGLARALQTKATQQGLKAAMLGQEDPPQHGLPRLLAAACQLQLNGNLQLELGEALAQERLLLPEDPLISGLLNSQALKACVDTALENLSTLKMKVAEVLAGEGHLYSRIPALLNTQPMLQLEYTATDRHPQALKDVQTKLQQHDVAQGQWNPSDPAPSSLGALDLLVCNCALATLGDPALALDNMVAALKEGGFLLVHTVLKGHALGETLACLPSEVQPAPSLLSQEEWESLFSRKALHLVGLKRSFYGTALFLCRRAIPQEKPIFLSVEDTSFQWVDSLKSTLATSSSQPVWLTAMDCPTSGVVGLVNCLRKEPGGHRIRCILLSNLSNTSHAPKLDPGSPELQQVLKHDLVMNVYRDGAWGAFRHFQLEQDKPKEQTAHAFVNVLTRGDLASIRWVSSPLKHTQPSSSGAQLCTVYYASLNFRDIMLATGKLSPDAIPGKWASRDCMLGMEFSGRDRCGRRVMGLVPAEGLATSVLLSSDFLWDVPSSWTLEEAASVPVVYTTAYYSLVVRGRIQRGETVLIHSGSGGVGQAAISIALSLGCRVFTTVGSAEKRAYLQARFPQLDDTSFANSRDTSFEQHVLLHTGGKGVDLVLNSLAEEKLQASVRCLAQHGRFLEIGKFDLSNNHPLGMAIFLKNVTFHGILLDALFEEANDSWREVAALLKAGIRDGVVKPLKCTVFPKAQVEDAFRYMAQGKHIGKVLVQVREEEPEAVLPGAQPTLISAISKTFCPAHKSYIITGGLGGFGLELARWLVLRGAQRLVLTSRSGIRTGYQAKHIREWRRQGIQVLVSTSNVSSLEGARALIAEATKLGPVGGVFNLAMVLRDAMLENQTPELFQDVNKPKYNGTLNLDRATREACPELDYFVAFSSVSCGRGNAGQTNYGFANSTMERICEQRRHDGLPGLAVQWGAIGDVGIVLEAMGTNDTVIGGTLPQRISSCMEVLDLFLNQPHAVLSSFVLAEKKAVAHGDGDTQRDLVKAVAHILGIRDLAGINLDSTLADLGLDSLMGVEVRQILEREHDLVLPMREVRQLTLRKLQEMSSKTDSATDTTAPKSRSDTSLKQNQAAAADTLLILGDSLSAGYRMSASAAWPALLNDKWQSKTSVVNASISGDTSQQGLARLPALLKQHQPRWVLVELGGNDGLRGFQPQQTEQTLRQILQDVKAANAEPLLMQIRLPANYGRRYNEAFSAIYPKLAKEFDVPLLPFFMEEVYLKPQWMQDDGIHPNRDAQPFIADWMAKQLQPLVNHDS

SEQ ID NO: 32 - protein, 2394 aa, synthetic construct
MEEVVIAGMSGKLPESENLQEFWANLIGGVDMVTDDDRRWKAGLYGLPKRSGKLKDLSKFDASFFGVHPKQAHTMDPQLRLLLEVSYEAIVDGGINPASLRGTNTGVWVGVSLSEASEALSRDPETLLGYSMVGCQRAMMANRLSFFFDFKGPSIALDTACSSSLLALQNAYQAIRSGECPAALVGGINLLLKPNTSVQFMKLGMLSPDGTCRSFDDSGSGYCRSEAVVAVLLTKKSLARRVYATILNAGTNTDGSKEQGVTFPSGEVQEQLICSLYQPAGLAPESLEYIEAHGTGTKVGDPQELNGITRSLCAFRQAPLLIGSTKSNMGHPEPASGLAALTKVLLSLEHGVWAPNLHFHNPNPEIPALLDGRLQVVDRPLPVRGGNVGINSFGFGGSNVHVILQPNTRQAPAPTAHAALPHLLHASGRTLEAVQDLLEQGRQHSQDLAFVSMLNDIAATPTAAMPFRGYTVLGVEGRVQEVQQVSTNKRPLWFICSGMGTQWRGMGLSLMRLDSFRESILRSDEAVKPLGVKVSDLLLSTDERTFDDIVHAFVSLTAIQIALIDLLTSVGLKPDGIIGHSLGEVACGYADGCLSQREAVLAAYWRGQCIKDAHLPPGSMAAVGLSWEECKQRCPAGVVPACHNSEDTVTISGPQAAVNEFVEQLKQEGVFAKEVRTGGLAFHSYFMEGIAPTLLQALKKVIREPRPRSARWLSTSIPEAQWQSSLARTSSAEYNVNNLVSPVLFQEALWHIPEHAVVLEIAPHALLQAVLKRGVKSSCTIIPLMKRDHKDNLEFFLTNLGKVHLTGINVNPNALFPPVEFPAPRGTPLISPHIKWDHSQTWDVPVAEDFPNGSSSSSATVYSIDASPESPDHYLVDHCIDGRVIFPGTGYLCLVWKTLARSLGLSLEETPVVFENVSFHQATILPKTGTVALEVRLLEASHAFEVSDTGNLIVSGKVYLWEDPNSKLFDHPEVPTPPESASVSRLTQGEVYKELRLRGYDYGPQFQGICEATLEGEQGKLLWKDNWVTFMDTMLQVSILGSSQQSLQLPTRVTAIYIDPATHRQKVYRLKEDTQVADVTTSRCLGITVSGGIHISRLQTTATSRRQQEQLVPTLEKFVFTPHMEAECLSESTALQKELQLCKGLARALQTKATQQGLKAAMLGQEDPPQHGLPRLLAAACQLQLNGNLQLELGEALAQERLLLPEDPLISGLLNSQALKACVDTALENLSTLKMKVAEVLAGEGHLYSRIPALLNTQPMLQLEYTATDRHPQALKDVQTKLQQHDVAQGQWNPSDPAPSSLGALDLLVCNCALATLGDPALALDNMVAALKEGGFLLVHTVLKGHALGETLACLPSEVQPAPSLLSQEEWESLFSRKALHLVGLKRSFYGTALFLCRRAIPQEKPIFLSVEDTSFQWVDSLKSTLATSSSQPVWLTAMDCPTSGVVGLVNCLRKEPGGHRIRCILLSNLSNTSHAPKLDPGSPELQQVLKHDLVMNVYRDGAWGAFRHFQLEQDKPKEQTAHAFVNVLTRGDLASIRWVSSPLKHTQPSSSGAQLCTVYYASLNFRDIMLATGKLSPDAIPGKWASRDCMLGMEFSGRDRCGRRVMGLVPAEGLATSVLLSSDFLWDVPSSWTLEEAASVPVVYTTAYYSLVVRGRIQRGETVLIHSGSGGVGQAAISIALSLGCRVFTTVGSAEKRAYLQARFPQLDDTSFANSRDTSFEQHVLLHTGGKGVDLVLNSLAEEKLQASVRCLAQHGRFLEIGKFDLSNNHPLGMAIFLKNVTFHGILLDALFEEANDSWREVAALLKAGIRDGVVKPLKCTVFPKAQVEDAFRYMAQGKHIGKVLVQVREEEPEAVLPGAQPTLISAISKTFCPAHKSYIITGGLGGFGLELARWLVLRGAQRLVLTSRSGIRTGYQAKHIREWRRQGIQVLVSTSNVSSLEGARALIAEATKLGPVGGVFNLAMVLRDAMLENQTPELFQDVNKPKYNGTLNLDRATREACPELDYFVAFSSVSCGRGNAGQTNYGFANSTMERICEQRRHDGLPGLAVQWGAIGDVGIVLEAMGTNDTVIGGTLPQRISSCMEVLDLFLNQPHAVLSSFVLAEKKAVAHGDGDTQRDLVKAVAHILGIRDLAGINLDSTLADLGLDSLMGVEVRQILEREHDLVLPMREVRQLTLRKLQEMSSKTDSATDTTAPKSRSDTSLKQNQAAAADTLLILGDSLSAGYRMSASAAWPALLNDKWQSKTSVVNASISGDTSQQGLARLPALLKQHQPRWVLVELGGNDGLRGFQPQQTEQTLRQILQDVKAANAEPLLMQIRLPANYGRRYNEAFSAIYPKLAKEFDVPLLPFFMEEVYLKPQWMQDDGIHPNRDAQPFIADWMAKQLQPLVNHDS

SEQ ID NO: 33 - protein, 2394 aa, synthetic construct
MEEVVIAGMSGKLPESENLQEFWANLIGGVDMVTDDDRRWKAGLYGLPKRSGKLKDLSKFDASFFGVHPKQAHTMDPQLRLLLEVSYEAIVDGGINPASLRGTNTGVWVGVSHSEASEALSRDPETLLGYSMVGCQRAMMANRLSFFFDFKGPSIALDTACSSSLLALQNAYQAIRSGECPAALVGGINLLLKPNTSVQFMKLGMLSPDGTCRSFDDSGSGYCRSEAVVAVLLTKKSLARRVYATILNAGTNTDGSKEQGVTFPSGEVQEQLICSLYQPAGLAPESLEYIEAHGTGTKVGDPQELNGITRSLCAFRQAPLLIGSTKSNMGHPEPASGLAALTKVLLSLEHGVWAPNLHFHNPNPEIPALLDGRLQVVDRPLPVRGGNVGINSFGFGGSNVHVILQPNTRQAPAPTAHAALPHLLHASGRTLEAVQDLLEQGRQHSQDLAFVSMLNDIAATPTAAMPFRGYTVLGVEGRVQEVQQVSTNKRPLWFICSGMGTQWRGMGLSLMRLDSFRESILRSDEAVKPLGVKVSDLLLSTDERTFDDIVHAFVSLTAIQIALIDLLTSVGLKPDGIIGHSLGEVACGYADGCLSQREAVLAAYWRGQCIKDAHLPPGSMAAVGLSWEECKQRCPAGVVPACHNSEDTVTISGPQAAVNEFVEQLKQEGVFAKEVRTGGLAFHSYFMEGIAPTLLQALKKVIREPRPRSARWLSTSIPEAQWQSSLARTSSAEYNVNNLVSPVLFQEALWHIPEHAVVLEIAPHALLQAVLKRGVKSSCTIIPLMKRDHKDNLEFFLTNLGKVHLTGINVNPNALFPPVEFPAPRGTPLISPHIKWDHSQTWDVPVAEDFPNGSSSSSATVYSIDASPESPDHYLVDHCIDGRVIFPGTGYLCLVWKTLARSLGLSLEETPVVFENVSFHQATILPKTGTVALEVRLLEASHAFEVSDTGNLIVSGKVYLWEDPNSKLFDHPEVPTPPESASVSRLTQGEVYKELRLRGYDYGPQFQGICEATLEGEQGKLLWKDNWVTFMDTMLQVSILGSSQQSLQLPTRVTAIYIDPATHRQKVYRLKEDTQVADVTTSRCLGITVSGGIHISRLQTTATSRRQQEQLVPTLEKFVFTPHMEAECLSESTALQKELQLCKGLARALQTKATQQGLKAAMLGQEDPPQHGLPRLLAAACQLQLNGNLQLELGEALAQERLLLPEDPLISGLLNSQALKACVDTALENLSTLKMKVAEVLAGEGHLYSRIPALLNTQPMLQLEYTATDRHPQALKDVQTKLQQHDVAQGQWNPSDPAPSSLGALDLLVCNCALATLGDPALALDNMVAALKEGGFLLVHTVLKGHALGETLACLPSEVQPAPSLLSQEEWESLFSRKALHLVGLKRSFYGTALFLCRRAIPQEKPIFLSVEDTSFQWVDSLKSTLATSSSQPVWLTAMDCPTSGVVGLVNCLRKEPGGHRIRCILLSNLSNTSHAPKLDPGSPELQQVLKHDLVMNVYRDGAWGAFRHFQLEQDKPKEQTAHAFVNVLTRGDLASIRWVSSPLKHTQPSSSGAQLCTVYYASLNFRDIMLATGKLSPDAIPGKWASRDCMLGMEFSGRDRCGRRVMGLVPAEGLATSVLLSSDFLWDVPSSWTLEEAASVPVVYTTAYYSLVVRGRIQRGETVLIHSGSGGVGQAAISIALSLGCRVFTTVGSAEKRAYLQARFPQLDDTSFANSRDTSFEQHVLLHTGGKGVDLVLNSLAEEKLQASVRCLAQHGRFLEIGKFDLSNNHPLGMAIFLKNVTFHGILLDALFEEANDSWREVAALLKAGIRDGVVKPLKCTVFPKAQVEDAFRYMAQGKHIGKVLVQVREEEPEAVLPGAQPTLISAISKTFCPAHKSYIITGGLGGFGLELARWLVLRGAQRLVLTSRSGIRTGYQAKHIREWRRQGIQVLVSTSNVSSLEGARALIAEATKLGPVGGVFNLAMVLRDAMLENQTPELFQDVNKPKYNGTLNLDRATREACPELDYFVAFSSVSCGRGNAGQTNYGFANSTMERICEQRRHDGLPGLAVQWGAIGDVGIVLEAMGTNDTVIGGTLPQRISSCMEVLDLFLNQPHAVLSSFVLAEKKAVAHGDGDTQRDLVKAVAHILGIRDLAGINLDSTLADLGLDSLMGVEVRQILEREHDLVLPMREVRQLTLRKLQEMSSKTDSATDTTAPKSRSDTSLKQNQAAAADTLLILGDSLSAGYRMSASAAWPALLNDKWQSKTSVVNASISGDTSQQGLARLPALLKQHQPRWVLVELGGNDGLRGFQPQQTEQTLRQILQDVKAANAEPLLMQIRLPANYGRRYNEAFSAIYPKLAKEFDVPLLPFFMEEVYLKPQWMQDDGIHPNRDAQPFIADWMAKQLQPLVNHDS

SEQ ID NO: 34 - protein, 2394 aa, synthetic construct
MEEVVIAGMSGKLPESENLQEFWANLIGGVDMVTDDDRRWKAGLYGLPKRSGKLKDLSKFDASFFGVHPKQAHTMDPQLRLLLEVSYEAIVDGGINPASLRGTNTGVWVGVSYSEASEALSRDPETLLGYSMVGCQRAMMANRLSFFFDFKGPSIALDTACSSSLLALQNAYQAIRSGECPAALVGGINLLLKPNTSVQFMKLGMLSPDGTCRSFDDSGSGYCRSEAVVAVLLTKKSLARRVYATILNAGTNTDGSKEQGVTFPSGEVQEQLICSLYQPAGLAPESLEYIEAHGTGTKVGDPQELNGITRSLCAFRQAPLLIGSTKSNMGHPEPASGLAALTKVLLSLEHGVWAPNLHFHNPNPEIPALLDGRLQVVDRPLPVRGGNVGINSFGFGGSNVHVILQPNTRQAPAPTAHAALPHLLHASGRTLEAVQDLLEQGRQHSQDLAFVSMLNDIAATPTAAMPFRGYTVLGVEGRVQEVQQVSTNKRPLWFICSGMGTQWRGMGLSLMRLDSFRESILRSDEAVKPLGVKVSDLLLSTDERTFDDIVHAFVSLTAIQIALIDLLTSVGLKPDGIIGHSLGEVACGYADGCLSQREAVLAAYWRGQCIKDAHLPPGSMAAVGLSWEECKQRCPAGVVPACHNSEDTVTISGPQAAVNEFVEQLKQEGVFAKEVRTGGLAFHSYFMEGIAPTLLQALKKVIREPRPRSARWLSTSIPEAQWQSSLARTSSAEYNVNNLVSPVLFQEALWHIPEHAVVLEIAPHALLQAVLKRGVKSSCTIIPLMKRDHKDNLEFFLTNLGKVHLTGINVNPNALFPPVEFPAPRGTPLISPHIKWDHSQTWDVPVAEDFPNGSSSSSATVYSIDASPESPDHYLVDHCIDGRVIFPGTGYLCLVWKTLARSLGLSLEETPVVFENVSFHQATILPKTGTVALEVRLLEASHAFEVSDTGNLIVSGKVYLWEDPNSKLFDHPEVPTPPESASVSRLTQGEVYKELRLRGYDYGPQFQGICEATLEGEQGKLLWKDNWVTFMDTMLQVSILGSSQQSLQLPTRVTAIYIDPATHRQKVYRLKEDTQVADVTTSRCLGITVSGGIHISRLQTTATSRRQQEQLVPTLEKFVFTPHMEAECLSESTALQKELQLCKGLARALQTKATQQGLKAAMLGQEDPPQHGLPRLLAAACQLQLNGNLQLELGEALAQERLLLPEDPLISGLLNSQALKACVDTALENLSTLKMKVAEVLAGEGHLYSRIPALLNTQPMLQLEYTATDRHPQALKDVQTKLQQHDVAQGQWNPSDPAPSSLGALDLLVCNCALATLGDPALALDNMVAALKEGGFLLVHTVLKGHALGETLACLPSEVQPAPSLLSQEEWESLFSRKALHLVGLKRSFYGTALFLCRRAIPQEKPIFLSVEDTSFQWVDSLKSTLATSSSQPVWLTAMDCPTSGVVGLVNCLRKEPGGHRIRCILLSNLSNTSHAPKLDPGSPELQQVLKHDLVMNVYRDGAWGAFRHFQLEQDKPKEQTAHAFVNVLTRGDLASIRWVSSPLKHTQPSSSGAQLCTVYYASLNFRDIMLATGKLSPDAIPGKWASRDCMLGMEFSGRDRCGRRVMGLVPAEGLATSVLLSSDFLWDVPSSWTLEEAASVPVVYTTAYYSLVVRGRIQRGETVLIHSGSGGVGQAAISIALSLGCRVFTTVGSAEKRAYLQARFPQLDDTSFANSRDTSFEQHVLLHTGGKGVDLVLNSLAEEKLQASVRCLAQHGRFLEIGKFDLSNNHPLGMAIFLKNVTFHGILLDALFEEANDSWREVAALLKAGIRDGVVKPLKCTVFPKAQVEDAFRYMAQGKHIGKVLVQVREEEPEAVLPGAQPTLISAISKTFCPAHKSYIITGGLGGFGLELARWLVLRGAQRLVLTSRSGIRTGYQAKHIREWRRQGIQVLVSTSNVSSLEGARALIAEATKLGPVGGVFNLAMVLRDAMLENQTPELFQDVNKPKYNGTLNLDRATREACPELDYFVAFSSVSCGRGNAGQTNYGFANSTMERICEQRRHDGLPGLAVQWGAIGDVGIVLEAMGTNDTVIGGTLPQRISSCMEVLDLFLNQPHAVLSSFVLAEKKAVAHGDGDTQRDLVKAVAHILGIRDLAGINLDSTLADLGLDSLMGVEVRQILEREHDLVLPMREVRQLTLRKLQEMSSKTDSATDTTAPKSRSDTSLKQNQAAAADTLLILGDSLSAGYRMSASAAWPALLNDKWQSKTSVVNASISGDTSQQGLARLPALLKQHQPRWVLVELGGNDGLRGFQPQQTEQTLRQILQDVKAANAEPLLMQIRLPANYGRRYNEAFSAIYPKLAKEFDVPLLPFFMEEVYLKPQWMQDDGIHPNRDAQPFIADWMAKQLQPLVNHDS

SEQ ID NO: 35 - protein, 293 aa, Mus musculus
LSTLLVNPEGPTLTQLNSVQSSERPLFLVHPIEGSTTVFHSLAAKLSVPTYGLQCTQAAPLDSIPNLAAYYIDCIKQVQPEGPYRIAGYSFGACVAFEMCSQLQAQQGPAPTHNNLFLFDGSHTYVLAYTQSYRAKMTPGCEAEAEAEALCFFIKQFLDVEHSKVLEALLPLKSLEDRVAASVDLITKSHHSLDRRELSFAAVSFYHKLRAADQYKPKAKYHGNVTLLRAKTGGTYGEDLGADYNLSQVCDGKVSVHIIEGDHRTLLEGSGLESIINIIHSSLAEPRVSVREG